European Patent Specification EP 3 826 662 B1, published September 11, 2024. Title: METHOD OF USING A GIP/GLP1 CO-AGONIST FOR DIABETES. Applicant: Eli Lilly and Company. The sequence listing filed with the application follows.

SEQUENCE LISTING (145 sequences)

SEQ ID NO: 1 - protein, 42 aa, Homo sapiens
YAEGTFISDYSIAMDKIHQQDFVNWLLAQKGKKNDWKHNITQ

SEQ ID NO: 2 - protein, 30 aa, Homo sapiens
  MOD_RES (30)..(30): AMIDATION
HAEGTFTSDVSSYLEGQAAKEFIAWLVKGR

SEQ ID NO: 3 - protein, 31 aa, Artificial Sequence
  Synthetic construct; Formula I
  VARIANT (1)..(1): Xaa at position 1 is selected from the group consisting of Y, H, D-Tyr, F, desH, and desY, or Xaa at position 1 and Xaa at position 2 combine to form desH-psi[NHCO]-Aib
  MOD_RES (1)..(1): The N-terminus of Xaa at position 1 is modified with R1, wherein the modification is selected from the group consisting of Ac and absent.
  VARIANT (2)..(2): Xaa at position 2 is selected from the group consisting of Aib, alpha-MeP, A, P, and D-Ala, or Xaa at position 1 combines with Xaa at position 2 to form desH-psi[NHCO]-Aib
  VARIANT (3)..(3): Xaa at position 3 is selected from the group of E, N, Aad, and cTA
  VARIANT (6)..(6): Xaa at position 6 is selected from the group consisting of F, alpha-MeF, and alpha-MeF(2F)
  VARIANT (10)..(10): Xaa at position 10 is selected from the group consisting of A, L, H, 3Pal, 4Pal, V, Y, E, alpha-MeF, alpha-MeF(2F), I, alpha-MeY, Q, D-His, D-Tyr, cTA, and K
  VARIANT (10)..(10): when Xaa at position 10 is K, then K is chemically modified by conjugation of the epsilon-amino group of the K side chain with (2-[2-(2-amino-ethoxy)-ethoxy]-acetyl)2-(gamma-Glu)-CO-(CH2)q-CO2 H
  MISC_FEATURE (10)..(31): When Xaa is K(2-[2-(2-amino-ethoxy)-ethoxy]-acetyl)2-(gamma-Glu)-CO-(CH2)q-CO 2H at positions 10, 12, 13, 14, 16, 17, 19, 20, 21, 23, 24, 26, 27, 28, 29, 30 or 31, q is 14, 15, 16, 17, 18, 19 or 20.
  VARIANT (11)..(11): Xaa at position 11 is selected from the group consisting of S, alpha-MeS, or D-Ser
  VARIANT (12)..(12): Xaa at position 12 is selected from the group consisting of I, S, D-Ile, and K
  MOD_RES (12)..(12): when Xaa at position 12 is K, then K is chemically modified by conjugation of the epsilon-amino group of the K side chain with (2-[2-(2-amino-ethoxy)-ethoxy]-acetyl)2-(gamma-Glu)-CO-(CH2)q-CO2 H
  VARIANT (13)..(13): Xaa at position 13 is selected from the group consisting of Nle, Aib, L, alpha-MeL, and K
  MOD_RES (13)..(13): when Xaa at position 13 is K, then K is chemically modified by conjugation of the epsilon-amino group of the K side chain with (2-[2-(2-amino-ethoxy)-ethoxy]-acetyl)2-(gamma-Glu)-CO-(CH2)q-CO2 H
  VARIANT (14)..(14): Xaa at position 14 is selected from the group consisting of L and K, wherein K is conjugated to a C16-C22 fatty acid wherein said fatty acid is optionally conjugated to said K via a linker
  VARIANT (16)..(16): Xaa at position 16 is selected from the group consisting of E, Orn, Dab, Dap, S, T, H, Aib, alpha-MeK, R, and K
  MOD_RES (16)..(16): when Xaa at position 16 is K, then K is optionally chemically modified by conjugation of the epsilon-amino group of the K side chain with (2-[2-(2-amino-ethoxy)-ethoxy]-acetyl)2 -(gamma-Glu)-CO-(CH2)q-CO2H
  VARIANT (17)..(17): Xaa at position 17 is selected from the group consisting of K, Q, I, and an amino acid conjugated to a C16-C22 fatty acid wherein said fatty acid is optionally conjugated to said amino acid via a linker
  VARIANT (19)..(19): Xaa at position 19 is selected from the group consisting of Q, A, and K
  MOD_RES (19)..(19): when Xaa at position 19 is K, then K is chemically modified by conjugation of the epsilon-amino group of the K side chain with (2-[2-(2-amino-ethoxy)-ethoxy]-acetyl)2 -(gamma-Glu)-CO-(CH2)q-CO2H
  VARIANT (20)..(20): Xaa at position 20 is selected from the group consisting of Aib, Q, H, R, K, and alpha-MeK
  MOD_RES (20)..(20): when Xaa at position 20 is K, then K  is optionally chemically modified by conjugation of the epsilon-amino group of the K side chain with (2-[2-(2-amino-ethoxy)-ethoxy]-acetyl)2 -(gamma-Glu)-CO-(CH2)q-CO2H
  VARIANT (21)..(21): Xaa at position 21 is selected from the group consisting of H, Aad, D, Aib, T, A, E, I, and K
  MOD_RES (21)..(21): when Xaa at position 21 is K, then K is chemically modified by conjugation of the epsilon-amino group of the K side chain with K(2-[2-(2-amino-ethoxy)-ethoxy]-acetyl)2-(gamma-Glu)-CO-(CH2)q-CO 2H
  VARIANT (22)..(22): Xaa at position 22 is selected from the group consisting of F and alpha-MeF
  VARIANT (23)..(23): Xaa at position 23 is selected from the group consisting of I, L, A, G, F, H, E, V, and  K
  MOD_RES (23)..(23): when Xaa at position 23 is K, then K is chemically modified by conjugation of the epsilon-amino group of the K side chain with K(2-[2-(2-amino-ethoxy)-ethoxy]-acetyl)2-(gamma-Glu)-CO-(CH2)q-CO 2H
  VARIANT (24)..(24): Xaa at position 24 is selected from the group consisting of S, Aad, D-Glu, E, Aib, H, V, A, Q, D, P, and K
  MOD_RES (24)..(24): when Xaa at position 24 is K, then K is chemically modified by conjugation of the epsilon-amino group of the K side chain with K(2-[2-(2-amino-ethoxy)-ethoxy]-acetyl)2-(gamma-Glu)-CO-(CH2)q-CO 2H
  VARIANT (25)..(25): Xaa at position 25 is selected from the group consisting of Y or alpha-MeY
  VARIANT (26)..(26): Xaa at position 26 is selected from the group consisting of L, alpha-MeL, and K
  MOD_RES (26)..(26): when Xaa at position 26 is K, then K is chemically modified by conjugation of the epsilon-amino group of the K side chain with (2-[2-(2-amino-ethoxy)-ethoxy]-acetyl)2-(gamma-Glu)-CO-(CH2)q-CO2 H
  VARIANT (27)..(27): Xaa at position 27 is selected from the group consisting of L, I, and K
  MOD_RES (27)..(27): when Xaa at position 27 is K, then K is chemically modified by conjugation of the epsilon-amino group of the K side chain with (2-[2-(2-amino-ethoxy)-ethoxy]-acetyl)2-(gamma-Glu)-CO-(CH2)q-CO2 H
  VARIANT (28)..(28): Xaa at position 28 is selected from the group consisting of E, A, S, D-Glu, and K
  MOD_RES (28)..(28): when Xaa at position 28 is K, then K is chemically modified by conjugation of the epsilon-amino group of the K side chain with (2-[2-(2-amino-ethoxy)-ethoxy]-acetyl)2-(gamma-Glu)-CO-(CH2)q-CO2 H
  VARIANT (29)..(29): Xaa at position 29 is selected from the group consisting of Aib, G, A, and K
  MOD_RES (29)..(29): when Xaa at position 29 is K, then K is chemically modified by conjugation of the epsilon-amino group of the K side chain with (2-[2-(2-amino-ethoxy)-ethoxy]-acetyl)2-(gamma-Glu)-CO-(CH2)q-CO2 H
  VARIANT (30)..(30): Xaa at position 30 is selected from the group consisting of C, G, G-R2, and K, wherein R2 is a modification of the C-terminal group, wherein the modification is NH2 or absent, wherein if X30 is G-R2, then X31 is absent.
  MOD_RES (30)..(30): when Xaa at position 30 is K, then K is chemically modified by conjugation of the epsilon-amino group of the K side chain with (2-[2-(2-amino-ethoxy)-ethoxy]-acetyl)2-(gamma-Glu)-CO-(CH2)q-CO2 H
  VARIANT (31)..(31): Xaa at position 31 is absent or is selected from the group consisting of SEQ ID NO:4, SEQ ID NO:5, SEQ ID:6, SEQ ID NO:7, SEQ ID NO:8, and SEQ ID NO:9
  MISC_FEATURE (31)..(31): wherein no more than one of X10, X12, X13, X14, X16, X17, X19, X20, X21, X23, X24, X26, X27, X28, X29, X30, X31, X32, X33, X34, X35, X36, X37, X38, X39, and X40 may be a substituent that contains a fatty acid
  MISC_FEATURE (31)..(31): wherein no more than one of X30, X34, X39, and X40 may be C
  MISC_FEATURE (31)..(31): wherein if one of X30, X34, X39, and X40 is C, then none of X10, X12, X13, X14, X16, X17, X19, X20, X21, X23, X24, X26, X27, X28, X29, X30, X31, X32, X33, X34, X35, X36, X37, X38, X39, and X40 is a substituent that contains a fatty acid
  MOD_RES (31)..(31): Xaa at position 31 is modified with R2, wherein the modification is NH2 to form a C-terminal amide or absent
XXXGTXTSDXXXXXDXXAXXXXXXXXXXXXX

SEQ ID NO: 4 - protein, 4 aa, Artificial Sequence
  Synthetic construct; SEQ ID NO:4 is PX32X33X34
  VARIANT (2)..(2): Xaa at position 2 is S or K, wherein K is chemically modified by conjugation of the epsilon-amino group of the K side chain with (2-[2-(2-amino-ethoxy)-ethoxy]-acetyl)2-(gamma-Glu)-CO-(CH2)q-CO2 H
  MISC_FEATURE (2)..(4): wherein q is selected from the group consisting of 14, 15, 16, 17, 18, 19, and 20.
  VARIANT (3)..(3): Xaa at position 3 is S or K, wherein K is chemically modified by conjugation of the epsilon-amino group of the K side chain with (2-[2-(2-amino-ethoxy)-ethoxy]-acetyl)2-(gamma-Glu)-CO-(CH2)q-CO2 H
  VARIANT (4)..(4): Xaa at position 4 is G, C or K, wherein K is chemically modified by conjugation of the epsilon-amino group of the K side chain with (2-[2-(2-amino-ethoxy)-ethoxy]-acetyl)2 -(gamma-Glu)-CO-(CH2)q-CO2H
  MOD_RES (4)..(4): The C-terminal group of Xaa at position 4 is modified with R2, wherein the modification is NH2 to form a C-terminal amide or absent
PXXX

SEQ ID NO: 5 - protein, 9 aa, Artificial Sequence
  Synthetic Construct; SEQ ID NO:5 is PX32X33X34X35X36X37X38X39
  VARIANT (2)..(2): Xaa at position 2 is S or K, wherein K is chemically modified by conjugation of the epsilon-amino group of the K side chain with (2-[2-(2-amino-ethoxy)-ethoxy]-acetyl)2-(gamma-Glu)-CO-(CH2)q-CO2 H
  MISC_FEATURE (2)..(9): wherein q is selected from the group consisting of 14, 15, 16, 17, 18, 19, and 20.
  VARIANT (3)..(3): Xaa at position 3 is S or K, wherein K is chemically modified by conjugation of the epsilon-amino group of the K side chain with (2-[2-(2-amino-ethoxy)-ethoxy]-acetyl)2-(gamma-Glu)-CO-(CH2)q-CO2 H
  VARIANT (4)..(4): Xaa at position 4 is G, C or K, wherein K is chemically modified by conjugation of the epsilon-amino group of the K side chain with (2-[2-(2-amino-ethoxy)-ethoxy]-acetyl)2 -(gamma-Glu)-CO-(CH2)q-CO2H
  VARIANT (5)..(5): Xaa at position 5 is A or K, wherein K is chemically modified by conjugation of the epsilon-amino group of the K side chain with (2-[2-(2-amino-ethoxy)-ethoxy]-acetyl)2-(gamma-Glu)-CO-(CH2)q-CO2 H
  VARIANT (6)..(6): Xaa at position 6 is P or K, wherein K is chemically modified by conjugation of the epsilon-amino group of the K side chain with (2-[2-(2-amino-ethoxy)-ethoxy]-acetyl)2-(gamma-Glu)-CO-(CH2)q-CO2 H
  VARIANT (7)..(7): Xaa at position 7 is P or K, wherein K is chemically modified by conjugation of the epsilon-amino group of the K side chain with (2-[2-(2-amino-ethoxy)-ethoxy]-acetyl)2-(gamma-Glu)-CO-(CH2)q-CO2 H
  VARIANT (8)..(8): Xaa at position 8 is P or K, wherein K is chemically modified by conjugation of the epsilon-amino group of the K side chain with (2-[2-(2-amino-ethoxy)-ethoxy]-acetyl)2-(gamma-Glu)-CO-(CH2)q-CO2 H
  VARIANT (9)..(9): Xaa at position 9 is C, S or K, wherein K is chemically modified by conjugation of the epsilon-amino group of the K side chain with (2-[2-(2-amino-ethoxy)-ethoxy]-acetyl)2 -(gamma-Glu)-CO-(CH2)q-CO2H
  MOD_RES (9)..(9): The C-terminal group of Xaa at position 9 is modified with R2, wherein the modification is NH2 to from a C-terminal amide or absent
PXXXXXXXX

SEQ ID NO: 6 - protein, 10 aa, Artificial Sequence
  Synthetic Construct; SEQ ID NO:6 is PX32X33X34X35X36X37X38X39X40
  VARIANT (2)..(2): Xaa at position 2 is S or K, wherein K is chemically modified by conjugation of the epsilon-amino group of the K side chain with (2-[2-(2-amino-ethoxy)-ethoxy]-acetyl)2-(gamma-Glu)-CO-(CH2)q-CO2 H
  MISC_FEATURE (2)..(10): wherein q is selected from the group consisting of 14, 15, 16, 17, 18, 19, and 20.
  VARIANT (3)..(3): Xaa at position 3 is S or K, wherein K is chemically modified by conjugation of the epsilon-amino group of the K side chain with (2-[2-(2-amino-ethoxy)-ethoxy]-acetyl)2-(gamma-Glu)-CO-(CH2)q-CO2 H
  VARIANT (4)..(4): Xaa at position 4 is G, C or K, wherein K is chemically modified by conjugation of the epsilon-amino group of the K side chain with (2-[2-(2-amino-ethoxy)-ethoxy]-acetyl)2 -(gamma-Glu)-CO-(CH2)q-CO2H
  VARIANT (5)..(5): Xaa at position 5 is A or K, wherein K is chemically modified by conjugation of the epsilon-amino group of the K side chain with (2-[2-(2-amino-ethoxy)-ethoxy]-acetyl)2-(gamma-Glu)-CO-(CH2)q-CO2 H
  VARIANT (6)..(6): Xaa at position 6 is P or K, wherein K is chemically modified by conjugation of the epsilon-amino group of the K side chain with (2-[2-(2-amino-ethoxy)-ethoxy]-acetyl)2-(gamma-Glu)-CO-(CH2)q-CO2 H
  VARIANT (7)..(7): Xaa at position 7 is P or K, wherein K is chemically modified by conjugation of the epsilon-amino group of the K side chain with K(2-[2-(2-amino-ethoxy)-ethoxy]-acetyl)2-(gamma-Glu)-CO-(CH2)q-CO 2H
  VARIANT (8)..(8): Xaa at position 8 is P or K, wherein K is chemically modified by conjugation of the epsilon-amino group of the K side chain with K(2-[2-(2-amino-ethoxy)-ethoxy]-acetyl)2-(gamma-Glu)-CO-(CH2)q-CO 2H
  VARIANT (9)..(9): Xaa at position 9 is C, S or K, wherein K is chemically modified by conjugation of the epsilon-amino group of the K side chain with (2-[2-(2-amino-ethoxy)-ethoxy]-acetyl)2 -(gamma-Glu)-CO-(CH2)q-CO2H
  VARIANT (10)..(10): Xaa at position 10 is C or K, wherein K is chemically modified by conjugation of the epsilon-amino group of the K side chain with (2-[2-(2-amino-ethoxy)-ethoxy]-acetyl)2-(gamma-Glu)-CO-(CH2)q-CO2 H
  MOD_RES (10)..(10): The C-terminal group of Xaa at position 10 is modified with R2, wherein the modification is NH2 to form a C-terminal amide or absent
PXXXXXXXXX

SEQ ID NO: 7 - protein, 4 aa, Artificial Sequence
  Synthetic Construct; SEQ ID NO:7 is K[(2-[2-(2-amino-ethoxy)-ethoxy]-acetyl)2-(gamma-Glu)-CO-(CH2)q-C O2 H]X32X33X34
  MOD_RES (1)..(1): K is chemically modified by conjugation of the epsilon-amino group of the K side chain with (2-[2-(2-amino-ethoxy)-ethoxy]-acetyl)2-(gamma-Glu)-CO-(CH2)q-CO2 H
  MISC_FEATURE (1)..(1): wherein q is selected from the group consisting of 14, 15, 16, 17, 18, 19, and 20
  VARIANT (2)..(2): Xaa at position 2 is S or K, wherein K is chemically modified by conjugation of the epsilon-amino group of the K side chain with (2-[2-(2-amino-ethoxy)-ethoxy]-acetyl)2-(gamma-Glu)-CO-(CH2)q-CO2 H
  VARIANT (3)..(3): Xaa at position 3 is S or K, wherein K is chemically modified by conjugation of the epsilon-amino group of the K side chain with (2-[2-(2-amino-ethoxy)-ethoxy]-acetyl)2-(gamma-Glu)-CO-(CH2)q-CO2 H
  VARIANT (4)..(4): Xaa at position 4 is G, C or K, wherein K is chemically modified by conjugation of the epsilon-amino group of the K side chain with (2-[2-(2-amino-ethoxy)-ethoxy]-acetyl)2 -(gamma-Glu)-CO-(CH2)q-CO2H
  MOD_RES (4)..(4): The C-terminal group of Xaa at position 4 is modified with R2, wherein the modification is NH2 to form a C-terminal amide or absent
KXXX

SEQ ID NO: 8 - protein, 9 aa, Artificial Sequence
  Synthetic Construct; SEQ ID NO:8 is K[(2-[2-(2-amino-ethoxy)-ethoxy]-acetyl)2-(gamma-Glu)-CO-(CH2)q-C O2H]X32X33X34X35X36X37X38X39
  MOD_RES (1)..(1): K is chemically modified by conjugation of the epsilon-amino group of the K side chain with (2-[2-(2-amino-ethoxy)-ethoxy]-acetyl)2-(gamma-Glu)-CO-(CH2)q-CO2 H
  MISC_FEATURE (1)..(1): wherein q is selected from the group consisting of 14, 15, 16, 17, 18, 19, and 20
  VARIANT (2)..(2): Xaa at position 2 is S or K, wherein K is chemically modified by conjugation of the epsilon-amino group of the K side chain with (2-[2-(2-amino-ethoxy)-ethoxy]-acetyl)2-(gamma-Glu)-CO-(CH2)q-CO2 H
  VARIANT (3)..(3): Xaa at position 3 is S or K, wherein K is chemically modified by conjugation of the epsilon-amino group of the K side chain with (2-[2-(2-amino-ethoxy)-ethoxy]-acetyl)2-(gamma-Glu)-CO-(CH2)q-CO2 H
  VARIANT (4)..(4): Xaa at position 4 is G, C or K, wherein K is chemically modified by conjugation of the epsilon-amino group of the K side chain with (2-[2-(2-amino-ethoxy)-ethoxy]-acetyl)2 -(gamma-Glu)-CO-(CH2)q-CO2H
  VARIANT (5)..(5): Xaa at position 5 is A or K, wherein K is chemically modified by conjugation of the epsilon-amino group of the K side chain with (2-[2-(2-amino-ethoxy)-ethoxy]-acetyl)2-(gamma-Glu)-CO-(CH2)q-CO2 H
  VARIANT (6)..(6): Xaa at position 6 is P or K, wherein K is chemically modified by conjugation of the epsilon-amino group of the K side chain with (2-[2-(2-amino-ethoxy)-ethoxy]-acetyl)2-(gamma-Glu)-CO-(CH2)q-CO2 H
  VARIANT (7)..(7): Xaa at position 7 is P or K, wherein K is chemically modified by conjugation of the epsilon-amino group of the K side chain with (2-[2-(2-amino-ethoxy)-ethoxy]-acetyl)2-(gamma-Glu)-CO-(CH2)q-CO2 H
  VARIANT (8)..(8): Xaa at position 8 is P or K, wherein K is chemically modified by conjugation of the epsilon-amino group of the K side chain with (2-[2-(2-amino-ethoxy)-ethoxy]-acetyl)2-(gamma-Glu)-CO-(CH2)q-CO2 H
  VARIANT (9)..(9): Xaa at position 9 is C, S or K, wherein K is chemically modified by conjugation of the epsilon-amino group of the K side chain with (2-[2-(2-amino-ethoxy)-ethoxy]-acetyl)2-(gamma-Glu)-CO-(CH2)q-CO2
  MOD_RES (9)..(9): The C-terminal group of Xaa at position 9 is modified with R2, wherein the modification is NH2 to form a C-terminal amide or absent
KXXXXXXXX

SEQ ID NO: 9 - protein, 10 aa, Artificial Sequence
  Synthetic Construct; SEQ ID NO:9 is K[(2-[2-(2-amino-ethoxy)-ethoxy]-acetyl)2-(gamma-Glu)-CO-(CH2)q-C O2H]X32X33X34X35X36X37X38X39X40
  MOD_RES (1)..(1): K is chemically modified by conjugation of the epsilon-amino group of the K side chain with (2-[2-(2-amino-ethoxy)-ethoxy]-acetyl)2-(gamma-Glu)-CO-(CH2)q-CO2 H
  MISC_FEATURE (1)..(1): wherein q is selected from the group consisting of 14, 15, 16, 17, 18, 19, and 20
  VARIANT (2)..(2): Xaa at position 2 is S or K, wherein K is chemically modified by conjugation of the epsilon-amino group of the K side chain with (2-[2-(2-amino-ethoxy)-ethoxy]-acetyl)2-(gamma-Glu)-CO-(CH2)q-CO2 H
  VARIANT (3)..(3): Xaa at position 3 is S or K, wherein K is chemically modified by conjugation of the epsilon-amino group of the K side chain with (2-[2-(2-amino-ethoxy)-ethoxy]-acetyl)2-(gamma-Glu)-CO-(CH2)q-CO2 H
  VARIANT (4)..(4): Xaa at position 4 is G, C or K, wherein K is chemically modified by conjugation of the epsilon-amino group of the K side chain with (2-[2-(2-amino-ethoxy)-ethoxy]-acetyl)2 -(gamma-Glu)-CO-(CH2)q-CO2H
  VARIANT (5)..(5): Xaa at position 5 is A or K, wherein K is chemically modified by conjugation of the epsilon-amino group of the K side chain with (2-[2-(2-amino-ethoxy)-ethoxy]-acetyl)2-(gamma-Glu)-CO-(CH2)q-CO2 H
  VARIANT (6)..(6): Xaa at position 6 is P or K, wherein K is chemically modified by conjugation of the epsilon-amino group of the K side chain with (2-[2-(2-amino-ethoxy)-ethoxy]-acetyl)2-(gamma-Glu)-CO-(CH2)q-CO2 H
  VARIANT (7)..(7): Xaa at position 7 is P or K, wherein K is chemically modified by conjugation of the epsilon-amino group of the K side chain with (2-[2-(2-amino-ethoxy)-ethoxy]-acetyl)2-(gamma-Glu)-CO-(CH2)q-CO2 H
  VARIANT (8)..(8): Xaa at position 8 is P or K, wherein K is chemically modified by conjugation of the epsilon-amino group of the K side chain with (2-[2-(2-amino-ethoxy)-ethoxy]-acetyl)2-(gamma-Glu)-CO-(CH2)q-CO2 H
  VARIANT (9)..(9): Xaa at position 9 is C, S or K, wherein K is chemically modified by conjugation of the epsilon-amino group of the K side chain with (2-[2-(2-amino-ethoxy)-ethoxy]-acetyl)2 -(gamma-Glu)-CO-(CH2)q-CO2H
  VARIANT (10)..(10): Xaa at position 10 is C or K, wherein K is chemically modified by conjugation of the epsilon-amino group of the K side chain with (2-[2-(2-amino-ethoxy)-ethoxy]-acetyl)2 -(gamma-Glu)-CO-(CH2)q-CO2H
  MOD_RES (10)..(10): The C-terminal group of Xaa at position 10 is modified with R2, wherein the modification is NH2 to form a C-terminal amide or absent
KXXXXXXXXX

SEQ ID NO: 10 - protein, 39 aa, Artificial Sequence
  Synthetic Construct
  MISC_FEATURE (2)..(2): Xaa at position 2 is Aib
  MISC_FEATURE (6)..(6): Xaa at position 6 is alpha-MeF(2F)
  MISC_FEATURE (13)..(13): Xaa at position 13 is alpha-MeL
  MOD_RES (17)..(17): K at position 17 is chemically modified by conjugation of the epsilon-amino group of the K side chain with (2-[2-(2-amino-ethoxy)-ethoxy]-acetyl)2-(gamma-Glu)-CO-(CH2)18-CO 2H
  MISC_FEATURE (20)..(20): Xaa at position 20 is Aib
  MISC_FEATURE (24)..(24): Xaa at position 24 is D-Glu
  MOD_RES (39)..(39): The Serine at position 39 is amidated
YXEGTXTSDYSIXLDEKAQXEFIXYLIEGGPSSGAPPPS

SEQ ID NO: 11 - protein, 39 aa, Artificial Sequence
  Synthetic Construct
  MISC_FEATURE (2)..(2): Xaa at position 2 is Aib
  MISC_FEATURE (6)..(6): Xaa at position 6 is alpha-MeF(2F)
  MISC_FEATURE (13)..(13): Xaa at position 13 is alpha-MeL
  MISC_FEATURE (16)..(16): Xaa at position 16 is Orn
  MOD_RES (17)..(17): K at position 17 is chemically modified by conjugation of the epsilon-amino group of the K side chain with (2-[2-(2-amino-ethoxy)-ethoxy]-acetyl)2-(gamma-Glu)-CO-(CH2)16-CO 2H
  MISC_FEATURE (20)..(20): Xaa at position 20 is Aib
  MISC_FEATURE (24)..(24): Xaa at position 24 is D-Glu
  MOD_RES (39)..(39): The Serine at position 39 is amidated
YXEGTXTSDYSIXLDXKAQXEFIXYLIEGGPSSGAPPPS

SEQ ID NO: 12 - protein, 39 aa, Artificial Sequence; identical to SEQ ID NO: 11
  Synthetic Construct
  MISC_FEATURE (2)..(2): Xaa at position 2 is Aib
  MISC_FEATURE (6)..(6): Xaa at position 6 is alpha-MeF(2F)
  MISC_FEATURE (13)..(13): Xaa at position 13 is alpha-MeL
  MISC_FEATURE (16)..(16): Xaa at position 16 is Orn
  MOD_RES (17)..(17): K at position 17 is chemically modified by conjugation of the epsilon-amino group of the K side chain with (2-[2-(2-amino-ethoxy)-ethoxy]-acetyl)2-(gamma-Glu)-CO-(CH2)18-CO 2H
  MISC_FEATURE (20)..(20): Xaa at position 20 is Aib
  MISC_FEATURE (24)..(24): Xaa at position 24 is D-Glu
  MISC_FEATURE (39)..(39): The Serine at position 39 is amidated

SEQ ID NO: 13 - protein, 39 aa, Artificial Sequence
  Synthetic Construct
  MISC_FEATURE (2)..(2): Xaa at position 2 is Aib
  MISC_FEATURE (6)..(6): Xaa at position 6 is alpha-MeF(2F)
  MISC_FEATURE (10)..(10): Xaa at position 10 is 4Pal
  MISC_FEATURE (13)..(13): Xaa at position 13 is alpha-MeL
  MISC_FEATURE (16)..(16): Xaa at position 16 is Orn
  MOD_RES (17)..(17): K at position 17 is chemically modified by conjugation of the epsilon-amino group of the K side chain with (2-[2-(2-amino-ethoxy)-ethoxy]-acetyl)2-(gamma-Glu)-CO-(CH2)16-CO 2H
  MISC_FEATURE (20)..(20): Xaa at position 20 is Aib
  MISC_FEATURE (24)..(24): Xaa at position 24 is D-Glu
  MISC_FEATURE (25)..(25): Xaa at position 25 is alpha-MeY
  MOD_RES (39)..(39): The Serine at position 39 is amidated
YXEGTXTSDXSIXLDXKAQXEFIXXLIEGGPSSGAPPPS

SEQ ID NO: 14 - protein, 39 aa, Artificial Sequence
  Synthetic Construct
  MISC_FEATURE (2)..(2): Xaa at position 2 is Aib
  MOD_RES (17)..(17): Lys at position 17 is chemically modified by conjugation of the epsilon-amino group of the Lys side chain with (2-[2-(2-amino-ethoxy)-ethoxy]-acetyl)2-(gamma-Glu)-CO-(CH2)18-CO 2H
  MISC_FEATURE (20)..(20): Xaa at position 20 is Aib
  MOD_RES (39)..(39): Ser at position 39 is amidated
YXEGTFTSDYSILLDKKAQXAFIEYLIEGGPSSGAPPPS

SEQ ID NO: 15 - protein, 39 aa, Artificial Sequence
  Synthetic Construct
  MISC_FEATURE (2)..(2): Xaa at position 2 is Aib
  MOD_RES (17)..(17): Lys at position 17 is chemically modified by conjugation of the epsilon-amino group of the Lys side chain with (2-[2-(2-amino-ethoxy)-ethoxy]-acetyl)2-(gamma-Glu)-CO-(CH2)18-CO 2H
  MISC_FEATURE (20)..(20): Xaa at position 20 is Aib
  MOD_RES (39)..(39): Ser at position 39 is amidated
YXEGTFTSDYSILLDSKAQXAFIEYLIEGGPSSGAPPPS

SEQ ID NO: 16 - protein, 39 aa, Artificial Sequence
  Synthetic Construct
  MISC_FEATURE (2)..(2): Xaa at position 2 is Aib
  MISC_FEATURE (13)..(13): Xaa at position 13 is alpha-methyl-Leu
  MOD_RES (17)..(17): Lys at position 17 is chemically modified by conjugation of the epsilon-amino group of the Lys side chain with (2-[2-(2-amino-ethoxy)-ethoxy]-acetyl)2-(gamma-Glu)-CO-(CH2)18-CO 2H
  MISC_FEATURE (20)..(20): Xaa at position 20 is Aib
  MOD_RES (39)..(39): Ser at position 39 is amidated
YXEGTFTSDYSIXLDKKAQXAFIEYLIEGGPSSGAPPPS

SEQ ID NO: 17 - protein, 39 aa, Artificial Sequence
  Synthetic Construct
  MISC_FEATURE (2)..(2): Xaa at position 2 is Aib
  MISC_FEATURE (13)..(13): Xaa at position 13 is alpha-methyl-Leu
  MOD_RES (17)..(17): Lys at position 17 is chemically modified by conjugation of the epsilon-amino group of the Lys side chain with (2-[2-(2-amino-ethoxy)-ethoxy]-acetyl)2-(gamma-Glu)-CO-(CH2)18-CO 2H
  MISC_FEATURE (20)..(20): Xaa at position 20 is alpha-methyl-Lys
  MOD_RES (39)..(39): Ser at position 39 is amidated
YXEGTFTSDYSIXLDEKAQXAFIEYLLEGGPSSGAPPPS

SEQ ID NO: 18 - protein, 39 aa, Artificial Sequence
  Synthetic Construct
  MISC_FEATURE (2)..(2): Xaa at position 2 is Aib
  MISC_FEATURE (13)..(13): Xaa at position 13 is alpha-methyl-Leu
  MOD_RES (17)..(17): Lys at position 17 is chemically modified by conjugation of the epsilon-amino group of the Lys side chain with (2-[2-(2-amino-ethoxy)-ethoxy]-acetyl)2-(gamma-Glu)-CO-(CH2)18-CO 2H
  MISC_FEATURE (20)..(20): Xaa at position 20 is alpha-methyl-Lys
  MISC_FEATURE (29)..(29): Xaa at position 29 is Aib
  MOD_RES (39)..(39): Ser at position 39 is amidated
YXEGTFTSDYSIXLDEKAQXAFIEYLLEXGPSSGAPPPS

SEQ ID NO: 19 - protein, 39 aa, Artificial Sequence
  Synthetic Construct
  MISC_FEATURE (2)..(2): Xaa at position 2 is Aib
  MOD_RES (12)..(12): Lys at position 12 is chemically modified by conjugation of the epsilon-amino group of the Lys side chain with (2-[2-(2-amino-ethoxy)-ethoxy]-acetyl)2-(gamma-Glu)-CO-(CH2)18-CO 2H
  MISC_FEATURE (20)..(20): Xaa at position 20 is Aib
  MOD_RES (39)..(39): Ser at position 39 is amidated
YXEGTFTSDYSKLLDKIAQXAFIEYLIEGGPSSGAPPPS

SEQ ID NO: 20 - protein, 39 aa, Artificial Sequence
  Synthetic Construct
  MISC_FEATURE (2)..(2): Xaa at position 2 is Aib
  MOD_RES (13)..(13): Lys at position 13 is chemically modified by conjugation of the epsilon-amino group of the Lys side chain with (2-[2-(2-amino-ethoxy)-ethoxy]-acetyl)2-(gamma-Glu)-CO-(CH2)18-CO 2H
  MISC_FEATURE (20)..(20): Xaa at position 20 is Aib
  MOD_RES (39)..(39): Ser at position 39 is amidated
YXEGTFTSDYSIKLDKIAQXAFIEYLIEGGPSSGAPPPS

SEQ ID NO: 21 - protein, 39 aa, Artificial Sequence
  Synthetic Construct
  MISC_FEATURE (2)..(2): Xaa at position 2 is Aib
  MOD_RES (16)..(16): Lys at position 16 is chemically modified by conjugation of the epsilon-amino group of the Lys side chain with (2-[2-(2-amino-ethoxy)-ethoxy]-acetyl)2-(gamma-Glu)-CO-(CH2)18-CO 2H
  MISC_FEATURE (20)..(20): Xaa at position 20 is Aib
  MOD_RES (39)..(39): Ser at position 39 is amidated
YXEGTFTSDYSILLDKIAQXAFIEYLIEGGPSSGAPPPS

SEQ ID NO: 22 - protein, 39 aa, Artificial Sequence
  Synthetic Construct
  MISC_FEATURE (2)..(2): Xaa at position 2 is Aib
  MOD_RES (19)..(19): Lys at position 19 is chemically modified by conjugation of the epsilon-amino group of the Lys side chain with (2-[2-(2-amino-ethoxy)-ethoxy]-acetyl)2-(gamma-Glu)-CO-(CH2)18-CO 2H
  MISC_FEATURE (20)..(20): Xaa at position 20 is Aib
  MOD_RES (39)..(39): Ser at position 39 is amidated
YXEGTFTSDYSILLDKIAKXAFIEYLIEGGPSSGAPPPS

SEQ ID NO: 23 - protein, 39 aa, Artificial Sequence
  Synthetic Construct
  MISC_FEATURE (2)..(2): Xaa at position 2 is Aib
  MISC_FEATURE (20)..(20): Xaa at position 20 is Aib
  MOD_RES (21)..(21): Lys at position 17 is chemically modified by conjugation of the epsilon-amino group of the Lys side chain with (2-[2-(2-amino-ethoxy)-ethoxy]-acetyl)2-(gamma-Glu)-CO-(CH2)18-CO 2H
  MOD_RES (39)..(39): Ser at position 39 is amidated
YXEGTFTSDYSILLDKIAQXKFIEYLIEGGPSSGAPPPS

SEQ ID NO: 24 - protein, 39 aa, Artificial Sequence
  Synthetic Construct
  MISC_FEATURE (2)..(2): Xaa at position 2 is Aib
  MISC_FEATURE (20)..(20): Xaa at position 20 is Aib
  MOD_RES (23)..(23): Lys at position 23 is chemically modified by conjugation of the epsilon-amino group of the Lys side chain with (2-[2-(2-amino-ethoxy)-ethoxy]-acetyl)2-(gamma-Glu)-CO-(CH2)18-CO 2H
  MOD_RES (39)..(39): Ser at position 39 is amidated
YXEGTFTSDYSILLDKIAQXAFKEYLIEGGPSSGAPPPS

SEQ ID NO: 25 - protein, 39 aa, Artificial Sequence
  Synthetic Construct
  MISC_FEATURE (2)..(2): Xaa at position 2 is Aib
  MISC_FEATURE (20)..(20): Xaa at position 20 is Aib
  MOD_RES (24)..(24): Lys at position 24 is chemically modified by conjugation of the epsilon-amino group of the Lys side chain with (2-[2-(2-amino-ethoxy)-ethoxy]-acetyl)2-(gamma-Glu)-CO-(CH2)18-CO 2H
  MOD_RES (39)..(39): Ser at position 39 is amidated
YXEGTFTSDYSILLDKIAQXAFIKYLIEGGPSSGAPPPS

SEQ ID NO: 26 - protein, 39 aa, Artificial Sequence
  Synthetic Construct
  MISC_FEATURE (2)..(2): Xaa at position 2 is Aib
  MISC_FEATURE (20)..(20): Xaa at position 20 is Aib
  MOD_RES (28)..(28): Lys at position 28 is chemically modified by conjugation of the epsilon-amino group of the Lys side chain with (2-[2-(2-amino-ethoxy)-ethoxy]-acetyl)2-(gamma-Glu)-CO-(CH2)18-CO 2H
  MOD_RES (39)..(39): Ser at position 39 is amidated
YXEGTFTSDYSILLDKIAQXAFIEYLIKGGPSSGAPPPS

SEQ ID NO: 27 - protein, 39 aa, Artificial Sequence
  Synthetic Construct
  MISC_FEATURE (2)..(2): Xaa at position 2 is Aib
  MISC_FEATURE (20)..(20): Xaa at position 20 is Aib
  MOD_RES (32)..(32): Lys at position 32 is chemically modified by conjugation of the epsilon-amino group of the Lys side chain with (2-[2-(2-amino-ethoxy)-ethoxy]-acetyl)2-(gamma-Glu)-CO-(CH2)18-CO 2H
  MOD_RES (39)..(39): Ser at position 39 is amidated
YXEGTFTSDYSILLDKIAQXAFIEYLIEGGPKSGAPPPS

SEQ ID NO: 28 - protein, 39 aa, Artificial Sequence
  Synthetic Construct
  MISC_FEATURE (2)..(2): Xaa at position 2 is Aib
  MISC_FEATURE (20)..(20): Xaa at position 20 is Aib
  MOD_RES (37)..(37): Lys at position 37 is chemically modified by conjugation of the epsilon-amino group of the Lys side chain with (2-[2-(2-amino-ethoxy)-ethoxy]-acetyl)2-(gamma-Glu)-CO-(CH2)18-CO 2H
  MOD_RES (39)..(39): Ser at position 39 is amidated
YXEGTFTSDYSILLDKIAQXAFIEYLIEGGPSSGAPKPS

SEQ ID NO: 29 - protein, 39 aa, Artificial Sequence
  Synthetic Construct
  MISC_FEATURE (2)..(2): Xaa at position 2 is Aib
  MISC_FEATURE (20)..(20): Xaa at position 20 is Aib
  MOD_RES (38)..(38): Lys at position 38 is chemically modified by conjugation of the epsilon-amino group of the Lys side chain with (2-[2-(2-amino-ethoxy)-ethoxy]-acetyl)2-(gamma-Glu)-CO-(CH2)18-CO 2H
  MOD_RES (39)..(39): Ser at position 39 is amidated
YXEGTFTSDYSILLDKIAQXAFIEYLIEGGPSSGAPPKS

SEQ ID NO: 30 - protein, 39 aa, Artificial Sequence
  Synthetic Construct
  MISC_FEATURE (2)..(2): Xaa at position 2 is Aib
  MISC_FEATURE (20)..(20): Xaa at position 20 is Aib
  MOD_RES (39)..(39): Lys at position 39 is chemically modified by conjugation of the epsilon-amino group of the Lys side chain with (2-[2-(2-amino-ethoxy)-ethoxy]-acetyl)2-(gamma-Glu)-CO-(CH2)18-CO 2H
  MOD_RES (39)..(39): Lys at position 39 is amidated
YXEGTFTSDYSILLDKIAQXAFIEYLIEGGPSSGAPPPK

SEQ ID NO: 31 - protein, 34 aa, Artificial Sequence
  Synthetic Construct
  MISC_FEATURE (2)..(2): Xaa at position 2 is Aib
  MOD_RES (17)..(17): Lys at position 17 is chemically modified by conjugation of the epsilon-amino group of the Lys side chain with (2-[2-(2-amino-ethoxy)-ethoxy]-acetyl)2-(gamma-Glu)-CO-(CH2)18-CO 2H
  MISC_FEATURE (20)..(20): Xaa at position 20 is Aib
  MOD_RES (34)..(34): Gly at position 34 is amidated
YXEGTFTSDYSILLDKKAQXAFIEYLIEGGPSSG

SEQ ID NO: 32 - protein, 30 aa, Artificial Sequence
  Synthetic Construct
  MISC_FEATURE (2)..(2): Xaa at position 2 is Aib
  MOD_RES (17)..(17): Lys at position 17 is chemically modified by conjugation of the epsilon-amino group of the Lys side chain with (2-[2-(2-amino-ethoxy)-ethoxy]-acetyl)2-(gamma-Glu)-CO-(CH2)18-CO 2H
  MISC_FEATURE (20)..(20): Xaa at position 20 is Aib
  MOD_RES (30)..(30): Gly at position 30 is amidated
YXEGTFTSDYSILLDKKAQXAFIEYLIEGG

SEQ ID NO: 33 - protein, 39 aa, Artificial Sequence
  Synthetic Construct
  MISC_FEATURE (2)..(2): Xaa at position 2 is Aib
  MISC_FEATURE (13)..(13): Xaa at position 13 is alpha-methyl-Leu
  MOD_RES (17)..(17): Lys at position 17 is chemically modified by conjugation of the epsilon-amino group of the Lys side chain with (2-[2-(2-amino-ethoxy)-ethoxy]-acetyl)2-(gamma-Glu)-CO-(CH2)18-CO 2H
  MISC_FEATURE (20)..(20): Xaa at position 20 is Aib
  MOD_RES (39)..(39): Ser at position 39 is amidated
YXEGTFTSDYSIXLDSKAQXAFIEYLIEGGPSSGAPPPS

SEQ ID NO: 34 - protein, 39 aa, Artificial Sequence
  Synthetic Construct
  MISC_FEATURE (2)..(2): Xaa at position 2 is Aib
  MISC_FEATURE (13)..(13): Xaa at position 13 is alpha-methyl-Leu
  MISC_FEATURE (16)..(16): Xaa at position 16 is Aib
  MOD_RES (17)..(17): Lys at position 17 is chemically modified by conjugation of the epsilon-amino group of the Lys side chain with (2-[2-(2-amino-ethoxy)-ethoxy]-acetyl)2-(gamma-Glu)-CO-(CH2)18-CO 2H
  MISC_FEATURE (20)..(20): Xaa at position 20 is Aib
  MOD_RES (39)..(39): Ser at position 39 is amidated
YXEGTFTSDYSIXLDXKAQXAFIEYLIEGGPSSGAPPPS

SEQ ID NO: 35 - protein, 30 aa, Artificial Sequence
  Synthetic Construct
  MISC_FEATURE (2)..(2): Xaa at position 2 is Aib
  MISC_FEATURE (13)..(13): Xaa at position 13 is alpha-methyl-Leu
  MOD_RES (17)..(17): Lys at position 17 is chemically modified by conjugation of the epsilon-amino group of the Lys side chain with (2-[2-(2-amino-ethoxy)-ethoxy]-acetyl)2-(gamma-Glu)-CO-(CH2)18-CO 2H
  MISC_FEATURE (20)..(20): Xaa at position 20 is Aib
  MOD_RES (30)..(30): Gly at position 30 is amidated
YXEGTFTSDYSIXLDKKAQXAFIEYLIEGG

SEQ ID NO: 36 - protein, 30 aa, Artificial Sequence
  Synthetic Construct
  MISC_FEATURE (2)..(2): Xaa at position 2 is Aib
  MISC_FEATURE (13)..(13): Xaa at position 13 is alpha-methyl-Leu
  MOD_RES (17)..(17): Lys at position 17 is chemically modified by conjugation of the epsilon-amino group of the Lys side chain with (2-[2-(2-amino-ethoxy)-ethoxy]-acetyl)2-(gamma-Glu)-CO-(CH2)18-CO 2H
  MISC_FEATURE (20)..(20): Xaa at position 20 is Aib
  MOD_RES (30)..(30): Gly at position 30 is amidated
YXEGTFTSDYSIXLDEKAQXAFIEYLIEGG

SEQ ID NO: 37 - protein, 30 aa, Artificial Sequence
  Synthetic Construct
  MISC_FEATURE (2)..(2): Xaa at position 2 is Aib
  MISC_FEATURE (13)..(13): Xaa at position 13 is alpha-methyl-Leu
  MOD_RES (17)..(17): Lys at position 17 is chemically modified by conjugation of the epsilon-amino group of the Lys side chain with (2-[2-(2-amino-ethoxy)-ethoxy]-acetyl)2-(gamma-Glu)-CO-(CH2)18-CO 2H
  MISC_FEATURE (20)..(20): Xaa at position 20 is Aib
  MOD_RES (30)..(30): Gly at position 30 is amidated
YXEGTFTSDYSIXLDSKAQXAFIEYLIEGG

SEQ ID NO: 38 - protein, 30 aa, Artificial Sequence
  Synthetic Construct
  MISC_FEATURE (2)..(2): Xaa at position 2 is Aib
  MISC_FEATURE (13)..(13): Xaa at position 13 is alpha-methyl-Leu
  MOD_RES (17)..(17): Lys at position 17 is chemically modified by conjugation of the epsilon-amino group of the Lys side chain with (2-[2-(2-amino-ethoxy)-ethoxy]-acetyl)2-(gamma-Glu)-CO-(CH2)18-CO 2H
  MISC_FEATURE (20)..(20): Xaa at position 20 is Aib
  MOD_RES (30)..(30): Gly at position 30 is amidated
YXEGTFTSDYSIXLDTKAQXAFIEYLIEGG

SEQ ID NO: 39 - protein, 39 aa, Artificial Sequence; identical to SEQ ID NO: 17
  Synthetic Construct
  MISC_FEATURE (2)..(2): Xaa at position 2 is Aib
  MISC_FEATURE (13)..(13): Xaa at position 13 is alpha-methyl-Leu
  MOD_RES (17)..(17): Lys at position 17 is chemically modified by conjugation of the epsilon-amino group of the Lys side chain with (2-[2-(2-amino-ethoxy)-ethoxy]-acetyl)2-(gamma-Glu)-CO-(CH2)18-CO 2H
  MISC_FEATURE (20)..(20): Xaa at position 20 is Aib
  MOD_RES (39)..(39): Ser at position 39 is amidated

SEQ ID NO: 40 - protein, 39 aa, Artificial Sequence
  Synthetic Construct
  MISC_FEATURE (2)..(2): Xaa at position 2 is Aib
  MISC_FEATURE (11)..(11): Xaa at position 11 is alpha-methyl-Ser
  MOD_RES (17)..(17): Lys at position 17 is chemically modified by conjugation of the epsilon-amino group of the Lys side chain with (2-[2-(2-amino-ethoxy)-ethoxy]-acetyl)2-(gamma-Glu)-CO-(CH2)18-CO 2H
  MISC_FEATURE (20)..(20): Xaa at position 20 is Aib
  MOD_RES (39)..(39): Ser at position 39 is amidated
YXEGTFTSDYXILLDKKAQXAFIEYLIEGGPSSGAPPPS

SEQ ID NO: 41 - protein, 39 aa, Artificial Sequence
  Synthetic Construct
  MISC_FEATURE (2)..(2): Xaa at position 2 is Aib
  MISC_FEATURE (6)..(6): Xaa at position 6 is alpha-methyl-Phe
  MISC_FEATURE (13)..(13): Xaa at position 13 is alpha-methyl-Leu
  MOD_RES (17)..(17): Lys at position 17 is chemically modified by conjugation of the epsilon-amino group of the Lys side chain with (2-[2-(2-amino-ethoxy)-ethoxy]-acetyl)2-(gamma-Glu)-CO-(CH2)18-CO 2H
  MISC_FEATURE (20)..(20): Xaa at position 20 is Aib
  MOD_RES (39)..(39): Ser at position 39 is amidated
YXEGTXTSDYSIXLDKKAQXAFIEYLIEGGPSSGAPPPS

SEQ ID NO: 42 - protein, 30 aa, Artificial Sequence
  Synthetic Construct
  MISC_FEATURE (2)..(2): Xaa at position 2 is Aib
  MISC_FEATURE (20)..(20): Xaa at position 20 is Aib
  MOD_RES (28)..(28): Lys at position 28 is chemically modified by conjugation of the epsilon-amino group of the Lys side chain with (2-[2-(2-amino-ethoxy)-ethoxy]-acetyl)2-(gamma-Glu)-CO-(CH2)18-CO 2H
  MOD_RES (30)..(30): Gly at position 30 is amidated
YXEGTFTSDYSILLDKIAQXAFIEYLIKGG

SEQ ID NO: 43 - protein, 39 aa, Artificial Sequence; identical to SEQ ID NO: 14
  Synthetic Construct
  MISC_FEATURE (2)..(2): Xaa at position 2 is D-Ala
  MOD_RES (17)..(17): Lys at position 17 is chemically modified by conjugation of the epsilon-amino group of the Lys side chain with (2-[2-(2-amino-ethoxy)-ethoxy]-acetyl)2-(gamma-Glu)-CO-(CH2)18-CO 2H
  MISC_FEATURE (20)..(20): Xaa at position 20 is Aib
  MOD_RES (39)..(39): Ser at position 39 is amidated

SEQ ID NO: 44 - protein, 39 aa, Artificial Sequence; identical to SEQ ID NO: 40
  Synthetic Construct
  MISC_FEATURE (2)..(2): Xaa at position 2 is Aib
  MISC_FEATURE (11)..(11): Xaa at position 11 is D-Ser
  MOD_RES (17)..(17): Lys at position 17 is chemically modified by conjugation of the epsilon-amino group of the Lys side chain with (2-[2-(2-amino-ethoxy)-ethoxy]-acetyl)2-(gamma-Glu)-CO-(CH2)18-CO 2H
  MISC_FEATURE (20)..(20): Xaa at position 20 is Aib
  MOD_RES (39)..(39): Ser at position 39 is amidated

SEQ ID NO: 45 - protein, 39 aa, Artificial Sequence
  Synthetic Construct
  MISC_FEATURE (2)..(2): Xaa at position 2 is Aib
  MOD_RES (17)..(17): Lys at position 17 is chemically modified by conjugation of the epsilon-amino group of the Lys side chain with (2-[2-(2-amino-ethoxy)-ethoxy]-acetyl)2-(gamma-Glu)-CO-(CH2)18-CO 2H
  MISC_FEATURE (20)..(20): Xaa at position 20 is Aib
  MISC_FEATURE (28)..(28): Xaa at position 28 is D-Glu
  MOD_RES (39)..(39): Ser at position 39 is amidated
YXEGTFTSDYSILLDKKAQXAFIEYLIXGGPSSGAPPPS

SEQ ID NO: 46 - protein, 39 aa, Artificial Sequence
  Synthetic Construct
  MISC_FEATURE (2)..(2): Xaa at position 2 is Aib
  MOD_RES (17)..(17): Lys at position 17 is chemically modified by conjugation of the epsilon-amino group of the Lys side chain with (2-[2-(2-amino-ethoxy)-ethoxy]-acetyl)2-(gamma-Glu)-CO-(CH2)18-CO 2H
  MISC_FEATURE (20)..(20): Xaa at position 20 is Aib
  MISC_FEATURE (24)..(24): Xaa at position 24 is D-Glu
  MOD_RES (39)..(39): Ser at position 39 is amidated
YXEGTFTSDYSILLDKKAQXAFIXYLIEGGPSSGAPPPS

SEQ ID NO: 47 - protein, 39 aa, Artificial Sequence
  Synthetic Construct
  MOD_RES (17)..(17): Lys at position 17 is chemically modified by conjugation of the epsilon-amino group of the Lys side chain with (2-[2-(2-amino-ethoxy)-ethoxy]-acetyl)2-(gamma-Glu)-CO-(CH2)18-CO 2H
  MISC_FEATURE (20)..(20): Xaa at position 20 is Aib
  MOD_RES (39)..(39): Ser at position 39 is amidated
YPEGTFTSDYSILLDKKAQXAFIEYLIEGGPSSGAPPPS

SEQ ID NO: 48 - protein, 39 aa, Artificial Sequence
  Synthetic Construct
  MISC_FEATURE (2)..(2): Xaa at position 2 is Aib
  MISC_FEATURE (3)..(3): Xaa at position 3 is Aad
  MOD_RES (17)..(17): Lys at position 17 is chemically modified by conjugation of the epsilon-amino group of the Lys side chain with (2-[2-(2-amino-ethoxy)-ethoxy]-acetyl)2-(gamma-Glu)-CO-(CH2)18-CO 2H
  MISC_FEATURE (20)..(20): Xaa at position 20 is Aib
  MOD_RES (39)..(39): Ser at position 39 is amidated
YXXGTFTSDYSILLDKKAQXAFIEYLIEGGPSSGAPPPS

SEQ ID NO: 49 - protein, 30 aa, Artificial Sequence
  Synthetic Construct
  MISC_FEATURE (2)..(2): Xaa at position 2 is Aib
  MISC_FEATURE (6)..(6): Xaa at position 6 is alpha-methyl-Phe
  MISC_FEATURE (20)..(20): Xaa at position 20 is Aib
  MOD_RES (28)..(28): Lys at position 28 is chemically modified by conjugation of the epsilon-amino group of the Lys side chain with (2-[2-(2-amino-ethoxy)-ethoxy]-acetyl)2-(gamma-Glu)-CO-(CH2)18-CO 2H
  MOD_RES (30)..(30): Gly at position 30 is amidated
YXEGTXTSDYSILLDKIAQXAFIEYLIKGG

SEQ ID NO: 50 - protein, 30 aa, Artificial Sequence
  Synthetic Construct
  MISC_FEATURE (2)..(2): Xaa at position 2 is Aib
  MISC_FEATURE (13)..(13): Xaa at position 13 is alpha-methyl-Leu
  MISC_FEATURE (20)..(20): Xaa at position 20 is Aib
  MOD_RES (28)..(28): Lys at position 28 is chemically modified by conjugation of the epsilon-amino group of the Lys side chain with (2-[2-(2-amino-ethoxy)-ethoxy]-acetyl)2-(gamma-Glu)-CO-(CH2)18-CO 2H
  MOD_RES (30)..(30): Gly at position 30 is amidated
YXEGTFTSDYSIXLDKIAQXAFIEYLIKGG

SEQ ID NO: 51 - protein, 30 aa, Artificial Sequence
  Synthetic Construct
  MISC_FEATURE (2)..(2): Xaa at position 2 is Aib
  MISC_FEATURE (6)..(6): Xaa at position 13 is alpha-methyl-Phe
  MOD_RES (17)..(17): Lys at position 17 is chemically modified by conjugation of the epsilon-amino group of the Lys side chain with (2-[2-(2-amino-ethoxy)-ethoxy]-acetyl)2-(gamma-Glu)-CO-(CH2)18-CO 2H
  MISC_FEATURE (20)..(20): Xaa at position 20 is Aib
  MOD_RES (30)..(30): Gly at position 30 is amidated
YXEGTXTSDYSILLDKKAQXAFIEYLIEGG

SEQ ID NO: 52 - protein, 30 aa, Artificial Sequence
  Synthetic Construct
  MISC_FEATURE (2)..(2): Xaa at position 2 is Aib
  MISC_FEATURE (6)..(6): Xaa at position 6 is alpha-methyl-Phe
  MISC_FEATURE (13)..(13): Xaa at position 13 is alpha-methyl-Leu
  MOD_RES (17)..(17): Lys at position 17 is chemically modified by conjugation of the epsilon-amino group of the Lys side chain with (2-[2-(2-amino-ethoxy)-ethoxy]-acetyl)2-(gamma-Glu)-CO-(CH2)18-CO 2H
  MISC_FEATURE (20)..(20): Xaa at position 20 is Aib
  MOD_RES (30)..(30): Gly at position 30 is amidated
YXEGTXTSDYSIXLDKKAQXAFIEYLIEGG

SEQ ID NO: 53 - protein, 30 aa, Artificial Sequence
  Synthetic Construct
  MISC_FEATURE (2)..(2): Xaa at position 2 is Aib
  MISC_FEATURE (6)..(6): Xaa at position 6 is alpha-methyl-Phe(2F)
  MISC_FEATURE (13)..(13): Xaa at position 13 is alpha-methyl-Leu
  MOD_RES (17)..(17): Lys at position 17 is chemically modified by conjugation of the epsilon-amino group of the Lys side chain with (2-[2-(2-amino-ethoxy)-ethoxy]-acetyl)2-(gamma-Glu)-CO-(CH2)18-CO 2H
  MISC_FEATURE (20)..(20): Xaa at position 20 is Aib
  MOD_RES (30)..(30): Gly at position 30 is amidated
YXEGTXTSDYSIXLDEKAQXEFIEYLIEGG

SEQ ID NO: 54 - protein, 30 aa, Artificial Sequence; identical to SEQ ID NO: 53
  Synthetic Construct
  MISC_FEATURE (2)..(2): Xaa at position 2 is Aib
  MISC_FEATURE (6)..(6): Xaa at position 6 is alpha-methyl-Phe(2F)
  MISC_FEATURE (13)..(13): Xaa at position 13 is alpha-methyl-Leu
  MOD_RES (17)..(17): Lys at position 17 is chemically modified by conjugation of the epsilon-amino group of the Lys side chain with (2-[2-(2-amino-ethoxy)-ethoxy]-acetyl)2-(gamma-Glu)-CO-(CH2)16-CO 2H
  MISC_FEATURE (20)..(20): Xaa at position 20 is Aib
  MOD_RES (30)..(30): Gly at position 30 is amidated

SEQ ID NO: 55 - protein, 39 aa, Artificial Sequence; identical to SEQ ID NO: 14
  Synthetic Construct
  MISC_FEATURE (2)..(2): Xaa at position 2 is Aib
  MOD_RES (17)..(17): Lys at position 17 is chemically modified by conjugation of the epsilon-amino group of the Lys side chain with (2-[2-(2-amino-ethoxy)-ethoxy]-acetyl)-AOC-(gamma-Glu)-CO-(CH2)18 -CO2H
  MISC_FEATURE (20)..(20): Xaa at position 20 is Aib
  MOD_RES (39)..(39): Ser at position 39 is amidated

SEQ ID NO: 56 - protein, 39 aa, Artificial Sequence; identical to SEQ ID NO: 14
  Synthetic Construct
  MISC_FEATURE (2)..(2): Xaa at position 2 is Aib
  MOD_RES (17)..(17): Lys at position 17 is chemically modified by conjugation of the epsilon-amino group of the Lys side chain with AOC-(2-[2-(2-amino-ethoxy)-ethoxy]-acetyl)-(gamma-Glu)-CO-(CH2)18 -CO2H
  MISC_FEATURE (20)..(20): Xaa at position 20 is Aib
  MOD_RES (39)..(39): Ser at position 39 is amidated

SEQ ID NO: 57 - protein, 39 aa, Artificial Sequence; identical to SEQ ID NO: 14
  Synthetic Construct
  MISC_FEATURE (2)..(2): Xaa at position 2 is Aib
  MOD_RES (17)..(17): Lys at position 17 is chemically modified by conjugation of the epsilon-amino group of the Lys side chain with (2-[2-(2-amino-ethoxy)-ethoxy]-acetyl)-(gamma-Glu)-(Trx)-CO-(CH2) 18-CO2H
  MISC_FEATURE (20)..(20): Xaa at position 20 is Aib
  MOD_RES (39)..(39): Ser at position 39 is amidated

SEQ ID NO: 58 - protein, 39 aa, Artificial Sequence; identical to SEQ ID NO: 14
  Synthetic Construct
  MISC_FEATURE (2)..(2): Xaa at position 2 is Aib
  MOD_RES (17)..(17): Lys at position 17 is chemically modified by conjugation of the epsilon-amino group of the Lys side chain with (2-[2-(2-amino-ethoxy)-ethoxy]-acetyl)-(Trx)-(gamma-Glu)-CO-(CH2) 18-CO2H
  MISC_FEATURE (20)..(20): Xaa at position 20 is Aib
  MOD_RES (39)..(39): Ser at position 39 is amidated

SEQ ID NO: 59 - protein, 39 aa, Artificial Sequence; identical to SEQ ID NO: 14
  Synthetic Construct
  MISC_FEATURE (2)..(2): Xaa at position 2 is Aib
  MOD_RES (17)..(17): Lys at position 17 is chemically modified by conjugation of the epsilon-amino group of the Lys side chain with (2-[2-(2-amino-ethoxy)-ethoxy]-acetyl)-(epsilon-Lys)-(gamma-Glu)- CO-(CH2)18-CO2H
  MISC_FEATURE (20)..(20): Xaa at position 20 is Aib
  MOD_RES (39)..(39): Ser at position 39 is amidated

SEQ ID NO: 60 - protein, 39 aa, Artificial Sequence; identical to SEQ ID NO: 14
  Synthetic Construct
  MISC_FEATURE (2)..(2): Xaa at position 2 is Aib
  MOD_RES (17)..(17): Lys at position 17 is chemically modified by conjugation of the epsilon-amino group of the Lys side chain with (2-[2-(2-amino-ethoxy)-ethoxy]-acetyl)2-(epsilon-Lys)-CO-(CH2)18- CO2H
  MISC_FEATURE (20)..(20): Xaa at position 20 is Aib
  MOD_RES (39)..(39): Ser at position 39 is amidated

SEQ ID NO: 61 - protein, 39 aa, Artificial Sequence; identical to SEQ ID NO: 14
  Synthetic Construct
  MISC_FEATURE (2)..(2): Xaa at position 2 is Aib
  MOD_RES (17)..(17): Lys at position 17 is chemically modified by conjugation of the epsilon-amino group of the Lys side chain with (2-[2-(2-amino-ethoxy)-ethoxy]-acetyl)-(epsilon-Lys)-(epsilon-Lys )-CO-(CH2)18-CO2H
  MISC_FEATURE (20)..(20): Xaa at position 2 is Aib
  MOD_RES (39)..(39): Ser at position 39 is amidated

SEQ ID NO: 62 - protein, 39 aa, Artificial Sequence
  Synthetic Construct
  MISC_FEATURE (2)..(2): Xaa at position 2 is Aib
  MISC_FEATURE (6)..(6): Xaa at position 6 is alpha-methyl-Phe
  MISC_FEATURE (13)..(13): Xaa at position 13 is alpha-methyl-Leu
  MOD_RES (17)..(17): Lys at position 17 is chemically modified by conjugation of the epsilon-amino group of the Lys side chain with (2-[2-(2-amino-ethoxy)-ethoxy]-acetyl)2-(gamma-Glu)-CO-(CH2)18-CO 2H
  MISC_FEATURE (20)..(20): Xaa at position 20 is Aib
  MOD_RES (39)..(39): Ser at position 39 is amidated
YXEGTXTSDYSIXLDEKAQXAFIEYLIEGGPSSGAPPPS

SEQ ID NO: 63 - protein, 39 aa, Artificial Sequence
  Synthetic Construct
  MISC_FEATURE (2)..(2): Xaa at position 2 is Aib
  MISC_FEATURE (6)..(6): Xaa at position 6 is alpha-methyl-Phe(2F)
  MISC_FEATURE (13)..(13): Xaa at position 13 is alpha-methyl-Leu
  MOD_RES (17)..(17): Lys at position 17 is chemically modified by conjugation of the epsilon-amino group of the Lys side chain with (2-[2-(2-amino-ethoxy)-ethoxy]-acetyl)2-(gamma-Glu)-CO-(CH2)18-CO 2H
  MISC_FEATURE (20)..(20): Xaa at position 20 is Aib
  MOD_RES (39)..(39): Ser at position 39 is amidated
YXEGTXTSDYSIXLDEKAQXEFIEYLIEGGPSSGAPPPS

SEQ ID NO: 64 - protein, 39 aa, Artificial Sequence
  Synthetic Construct
  MISC_FEATURE (2)..(2): Xaa at position 2 is Aib
  MISC_FEATURE (3)..(3): Xaa at position 3 is cTA
  MISC_FEATURE (6)..(6): Xaa at position 6 is alpha-methyl-Phe
  MISC_FEATURE (13)..(13): Xaa at position 13 is alpha-methyl-Leu
  MOD_RES (17)..(17): Lys at position 17 is chemically modified by conjugation of the epsilon-amino group of the Lys side chain with (2-[2-(2-amino-ethoxy)-ethoxy]-acetyl)2-(gamma-Glu)-CO-(CH2)18-CO 2H
  MISC_FEATURE (20)..(20): Xaa at position 20 is Aib
  MOD_RES (39)..(39): Ser at position 39 is amidated
YXXGTXTSDYSIXLDEKAQXAFIEYLIEGGPSSGAPPPS

SEQ ID NO: 65 - protein, 34 aa, Artificial Sequence
  Synthetic Construct
  MISC_FEATURE (2)..(2): Xaa at position 2 is Aib
  MISC_FEATURE (6)..(6): Xaa at position 6 is alpha-methyl-Phe
  MISC_FEATURE (13)..(13): Xaa at position 13 is alpha-methyl-Leu
  MOD_RES (17)..(17): Lys at position 17 is chemically modified by conjugation of the epsilon-amino group of the Lys side chain with (2-[2-(2-amino-ethoxy)-ethoxy]-acetyl)2-(gamma-Glu)-CO-(CH2)18-CO 2H
  MISC_FEATURE (20)..(20): Xaa at position 20 is Aib
  MOD_RES (34)..(34): Gly at position 34 is amidated
YXEGTXTSDYSIXLDKKAQXEFIEYLIEGGPSSG

SEQ ID NO: 66 - protein, 39 aa, Artificial Sequence; identical to SEQ ID NO: 41
  Synthetic Construct
  MISC_FEATURE (2)..(2): Xaa at position 2 is Aib
  MISC_FEATURE (6)..(6): Xaa at position 6 is alpha-methyl-Phe
  MISC_FEATURE (13)..(13): Xaa at position 13 is alpha-methyl-Leu
  MOD_RES (17)..(17): Lys at position 17 is chemically modified by conjugation of the epsilon-amino group of the Lys side chain with (2-[2-(2-amino-ethoxy)-ethoxy]-acetyl)2-(gamma-Glu)2-CO-(CH2)18-C O2H
  MISC_FEATURE (20)..(20): Xaa at position 20 is Aib
  MOD_RES (39)..(39): Ser at position 39 is amidated

SEQ ID NO: 67 - protein, 39 aa, Artificial Sequence
  Synthetic Construct
  MISC_FEATURE (2)..(2): Xaa at position 2 is Aib
  MISC_FEATURE (6)..(6): Xaa at position 6 is alpha-methyl-Phe
  MISC_FEATURE (13)..(13): Xaa at position 13 is alpha-methyl-Leu
  MOD_RES (17)..(17): Lys at position 17 is chemically modified by conjugation of the epsilon-amino group of the Lys side chain with (2-[2-(2-amino-ethoxy)-ethoxy]-acetyl)2-(gamma-Glu)-CO-(CH2)18-CO 2H
  MISC_FEATURE (20)..(20): Xaa at position 20 is Aib
  MOD_RES (39)..(39): Ser at position 39 is amidated
YXEGTXTSDYSIXLDKKAQXAFIEYLIEAGPSSGAPPPS

SEQ ID NO: 68 - protein, 39 aa, Artificial Sequence
  Synthetic Construct
  MISC_FEATURE (2)..(2): Xaa at position 2 is Aib
  MISC_FEATURE (6)..(6): Xaa at position 6 is alpha-methyl-Phe
  MOD_RES (17)..(17): Lys at position 17 is chemically modified by conjugation of the epsilon-amino group of the Lys side chain with (2-[2-(2-amino-ethoxy)-ethoxy]-acetyl)2-(gamma-Glu)-CO-(CH2)18-CO 2H
  MISC_FEATURE (20)..(20): Xaa at position 20 is Aib
  MOD_RES (39)..(39): Ser at position 39 is amidated
YXEGTXTSDHSILLDKKAQXAFIEYLIEGGPSSGAPPPS

SEQ ID NO: 69 - protein, 39 aa, Artificial Sequence
  Synthetic Construct
  MISC_FEATURE (2)..(2): Xaa at position 2 is Aib
  MISC_FEATURE (6)..(6): Xaa at position 6 is alpha-methyl-Phe
  MOD_RES (17)..(17): Lys at position 17 is chemically modified by conjugation of the epsilon-amino group of the Lys side chain with (2-[2-(2-amino-ethoxy)-ethoxy]-acetyl)2-(gamma-Glu)-CO-(CH2)18-CO 2H
  MISC_FEATURE (20)..(20): Xaa at position 20 is Aib
  MOD_RES (39)..(39): Ser at position 39 is amidated
YXEGTXTSDLSILLDKKAQXAFIEYLIEGGPSSGAPPPS

SEQ ID NO: 70 - protein, 39 aa, Artificial Sequence
  Synthetic Construct
  MISC_FEATURE (2)..(2): Xaa at position 2 is Aib
  MISC_FEATURE (6)..(6): Xaa at position 6 is alpha-methyl-Phe
  MISC_FEATURE (13)..(13): Xaa at position 13 is alpha-methyl-Leu
  MOD_RES (17)..(17): Lys at position 17 is chemically modified by conjugation of the epsilon-amino group of the Lys side chain with (2-[2-(2-amino-ethoxy)-ethoxy]-acetyl)2-(gamma-Glu)-CO-(CH2)18-CO 2H
  MISC_FEATURE (20)..(20): Xaa at position 20 is Aib
  MISC_FEATURE (21)..(21): Xaa at position 21 is Aad
  MOD_RES (39)..(39): Ser at position 39 is amidated
YXEGTXTSDYSIXLDKKAQXXFIEYLIEGGPSSGAPPPS

SEQ ID NO: 71 - protein, 39 aa, Artificial Sequence
  Synthetic Construct
  MISC_FEATURE (2)..(2): Xaa at position 2 is Aib
  MISC_FEATURE (6)..(6): Xaa at position 6 is alpha-methyl-Phe
  MISC_FEATURE (13)..(13): Xaa at position 13 is alpha-methyl-Leu
  MOD_RES (17)..(17): Lys at position 17 is chemically modified by conjugation of the epsilon-amino group of the Lys side chain with (2-[2-(2-amino-ethoxy)-ethoxy]-acetyl)2-(gamma-Glu)-CO-(CH2)18-CO 2H
  MISC_FEATURE (20)..(20): Xaa at position 20 is Aib
  MOD_RES (39)..(39): Ser at position 39 is amidated
YXEGTXTSDYSIXLDKKAQXTFIEYLIEGGPSSGAPPPS

SEQ ID NO: 72 - protein, 39 aa, Artificial Sequence
  Synthetic Construct
  MISC_FEATURE (2)..(2): Xaa at position 2 is Aib
  MISC_FEATURE (6)..(6): Xaa at position 6 is alpha-methyl-Phe
  MISC_FEATURE (13)..(13): Xaa at position 13 is alpha-methyl-Leu
  MOD_RES (17)..(17): Lys at position 17 is chemically modified by conjugation of the epsilon-amino group of the Lys side chain with (2-[2-(2-amino-ethoxy)-ethoxy]-acetyl)2-(gamma-Glu)-CO-(CH2)18-CO 2H
  MISC_FEATURE (20)..(20): Xaa at position 20 is Aib
  MOD_RES (39)..(39): Ser at position 39 is amidated
YXEGTXTSDYSIXLDKKAQXDFIEYLIEGGPSSGAPPPS

SEQ ID NO: 73 - protein, 39 aa, Artificial Sequence; identical to SEQ ID NO: 70
  Synthetic Construct
  MISC_FEATURE (2)..(2): Xaa at position 2 is Aib
  MISC_FEATURE (6)..(6): Xaa at position 6 is alpha-methyl-Phe
  MISC_FEATURE (13)..(13): Xaa at position 13 is alpha-methyl-Leu
  MOD_RES (17)..(17): Lys at position 17 is chemically modified by conjugation of the epsilon-amino group of the Lys side chain with (2-[2-(2-amino-ethoxy)-ethoxy]-acetyl)2-(gamma-Glu)-CO-(CH2)18-CO 2H
  MISC_FEATURE (20)..(20): Xaa at position 20 is Aib
  MISC_FEATURE (21)..(21): Xaa at position 21 is Aib
  MOD_RES (39)..(39): Ser at position 39 is amidated

SEQ ID NO: 74 - protein, 39 aa, Artificial Sequence
  Synthetic Construct
  MISC_FEATURE (2)..(2): Xaa at position 2 is Aib
  MISC_FEATURE (6)..(6): Xaa at position 6 is alpha-methyl-Phe
  MISC_FEATURE (13)..(13): Xaa at position 13 is alpha-methyl-Leu
  MOD_RES (17)..(17): Lys at position 17 is chemically modified by conjugation of the epsilon-amino group of the Lys side chain with (2-[2-(2-amino-ethoxy)-ethoxy]-acetyl)2-(gamma-Glu)-CO-(CH2)18-CO 2H
  MISC_FEATURE (21)..(21): Xaa at position 21 is Aib
  MOD_RES (39)..(39): Ser at position 39 is amidated
YXEGTXTSDYSIXLDKKAQHXFIEYLIEGGPSSGAPPPS

SEQ ID NO: 75 - protein, 39 aa, Artificial Sequence; identical to SEQ ID NO: 10
  Synthetic Construct
  MISC_FEATURE (2)..(2): Xaa at position 2 is Aib
  MISC_FEATURE (6)..(6): Xaa at position 6 is alpha-methyl-Phe(2F)
  MISC_FEATURE (13)..(13): Xaa at position 13 is alpha-methyl-Leu
  MOD_RES (17)..(17): Lys at position 17 is chemically modified by conjugation of the epsilon-amino group of the Lys side chain with (2-[2-(2-amino-ethoxy)-ethoxy]-acetyl)2-(gamma-Glu)-CO-(CH2)18-CO 2H
  MISC_FEATURE (20)..(20): Xaa at position 20 is Aib
  MISC_FEATURE (24)..(24): Xaa at position 24 is Aad
  MOD_RES (39)..(39): Ser at position 39 is amidated

SEQ ID NO: 76 - protein, 39 aa, Artificial Sequence
  Synthetic Construct
  MISC_FEATURE (2)..(2): Xaa at position 2 is Aib
  MISC_FEATURE (6)..(6): Xaa at position 6 is alpha-methyl-Phe(2F)
  MISC_FEATURE (13)..(13): Xaa at position 13 is alpha-methyl-Leu
  MOD_RES (17)..(17): Lys at position 17 is chemically modified by conjugation of the epsilon-amino group of the Lys side chain with (2-[2-(2-amino-ethoxy)-ethoxy]-acetyl)2-(gamma-Glu)-CO-(CH2)18-CO 2H
  MISC_FEATURE (20)..(20): Xaa at position 20 is Aib
  MOD_RES (39)..(39): Ser at position 39 is amidated
YXEGTXTSDYSIXLDEKAQXEFIAYLIEGGPSSGAPPPS

SEQ ID NO: 77 - protein, 39 aa, Artificial Sequence
  Synthetic Construct
  MISC_FEATURE (2)..(2): Xaa at position 2 is Aib
  MISC_FEATURE (6)..(6): Xaa at position 6 is alpha-methyl-Phe(2F)
  MISC_FEATURE (13)..(13): Xaa at position 13 is alpha-methyl-Leu
  MOD_RES (17)..(17): Lys at position 17 is chemically modified by conjugation of the epsilon-amino group of the Lys side chain with (2-[2-(2-amino-ethoxy)-ethoxy]-acetyl)2-(gamma-Glu)-CO-(CH2)18-CO 2H
  MISC_FEATURE (20)..(20): Xaa at position 20 is Aib
  MOD_RES (39)..(39): Ser at position 39 is amidated
YXEGTXTSDYSIXLDEKAQXEFIVYLIEGGPSSGAPPPS

SEQ ID NO: 78 - protein, 39 aa, Artificial Sequence
  Synthetic Construct
  MISC_FEATURE (2)..(2): Xaa at position 2 is Aib
  MISC_FEATURE (6)..(6): Xaa at position 6 is alpha-methyl-Phe(2F)
  MISC_FEATURE (13)..(13): Xaa at position 13 is alpha-methyl-Leu
  MOD_RES (17)..(17): Lys at position 17 is chemically modified by conjugation of the epsilon-amino group of the Lys side chain with (2-[2-(2-amino-ethoxy)-ethoxy]-acetyl)2-(gamma-Glu)-CO-(CH2)18-CO 2H
  MISC_FEATURE (20)..(20): Xaa at position 20 is Aib
  MOD_RES (39)..(39): Ser at position 39 is amidated
YXEGTXTSDYSIXLDEKAQXEFISYLIEGGPSSGAPPPS

SEQ ID NO: 79 - protein, 39 aa, Artificial Sequence
  Synthetic Construct
  MISC_FEATURE (2)..(2): Xaa at position 2 is Aib
  MISC_FEATURE (6)..(6): Xaa at position 6 is alpha-methyl-Phe(2F)
  MISC_FEATURE (13)..(13): Xaa at position 13 is alpha-methyl-Leu
  MOD_RES (17)..(17): Lys at position 17 is chemically modified by conjugation of the epsilon-amino group of the Lys side chain with (2-[2-(2-amino-ethoxy)-ethoxy]-acetyl)2-(gamma-Glu)-CO-(CH2)18-CO 2H
  MISC_FEATURE (20)..(20): Xaa at position 20 is Aib
  MOD_RES (39)..(39): Ser at position 39 is amidated
YXEGTXTSDYSIXLDEKAQXEFIPYLIEGGPSSGAPPPS

SEQ ID NO: 80 - protein, 39 aa, Artificial Sequence; identical to SEQ ID NO: 10
  Synthetic Construct
  MISC_FEATURE (2)..(2): Xaa at position 2 is Aib
  MISC_FEATURE (6)..(6): Xaa at position 6 is alpha-methyl-Phe(2F)
  MISC_FEATURE (13)..(13): Xaa at position 13 is alpha-methyl-Leu
  MOD_RES (17)..(17): Lys at position 17 is chemically modified by conjugation of the epsilon-amino group of the Lys side chain with (2-[2-(2-amino-ethoxy)-ethoxy]-acetyl)2-(gamma-Glu)-CO-(CH2)18-CO 2H
  MISC_FEATURE (20)..(20): Xaa at position 20 is Aib
  MISC_FEATURE (24)..(24): Xaa at position 24 is Aib
  MOD_RES (39)..(39): Ser at position 39 is amidated

SEQ ID NO: 81 - protein, 39 aa, Artificial Sequence
  Synthetic Construct
  MISC_FEATURE (2)..(2): Xaa at position 2 is Aib
  MISC_FEATURE (6)..(6): Xaa at position 6 is alpha-methyl-Phe(2F)
  MISC_FEATURE (13)..(13): Xaa at position 13 is alpha-methyl-Leu
  MOD_RES (17)..(17): Lys at position 17 is chemically modified by conjugation of the epsilon-amino group of the Lys side chain with (2-[2-(2-amino-ethoxy)-ethoxy]-acetyl)2-(gamma-Glu)-CO-(CH2)18-CO 2H
  MISC_FEATURE (20)..(20): Xaa at position 20 is Aib
  MOD_RES (39)..(39): Ser at position 39 is amidated
YXEGTXTSDYSIXLDEKAQXEFIHYLIEGGPSSGAPPPS

SEQ ID NO: 82 - protein, 39 aa, Artificial Sequence
  Synthetic Construct
  MISC_FEATURE (2)..(2): Xaa at position 2 is Aib
  MISC_FEATURE (6)..(6): Xaa at position 6 is alpha-methyl-Phe(2F)
  MISC_FEATURE (13)..(13): Xaa at position 13 is alpha-methyl-Leu
  MOD_RES (17)..(17): Lys at position 17 is chemically modified by conjugation of the epsilon-amino group of the Lys side chain with (2-[2-(2-amino-ethoxy)-ethoxy]-acetyl)2-(gamma-Glu)-CO-(CH2)18-CO 2H
  MISC_FEATURE (20)..(20): Xaa at position 20 is Aib
  MOD_RES (39)..(39): Ser at position 39 is amidated
YXEGTXTSDHSIXLDEKAQXEFIEYLIEGGPSSGAPPPS

SEQ ID NO: 83 - protein, 39 aa, Artificial Sequence
  Synthetic Construct
  MISC_FEATURE (2)..(2): Xaa at position 2 is Aib
  MISC_FEATURE (6)..(6): Xaa at position 6 is alpha-methyl-Phe(2F)
  MISC_FEATURE (10)..(10): Xaa at position 10 is cTA
  MISC_FEATURE (13)..(13): Xaa at position 13 is alpha-methyl-Leu
  MOD_RES (17)..(17): Lys at position 17 is chemically modified by conjugation of the epsilon-amino group of the Lys side chain with (2-[2-(2-amino-ethoxy)-ethoxy]-acetyl)2-(gamma-Glu)-CO-(CH2)18-CO 2H
  MISC_FEATURE (20)..(20): Xaa at position 20 is Aib
  MOD_RES (39)..(39): Ser at position 39 is amidated
YXEGTXTSDXSIXLDEKAQXEFIEYLIEGGPSSGAPPPS

SEQ ID NO: 84 - protein, 39 aa, Artificial Sequence; identical to SEQ ID NO: 83
  Synthetic Construct
  MISC_FEATURE (2)..(2): Xaa at position 2 is Aib
  MISC_FEATURE (6)..(6): Xaa at position 6 is alpha-methyl-Phe(2F)
  MISC_FEATURE (10)..(10): Xaa at position 10 is 3Pal
  MISC_FEATURE (13)..(13): Xaa at position 13 is alpha-methyl-Leu
  MOD_RES (17)..(17): Lys at position 17 is chemically modified by conjugation of the epsilon-amino group of the Lys side chain with (2-[2-(2-amino-ethoxy)-ethoxy]-acetyl)2-(gamma-Glu)-CO-(CH2)18-CO 2H
  MISC_FEATURE (20)..(20): Xaa at position 20 is Aib
  MOD_RES (39)..(39): Ser at position 39 is amidated

SEQ ID NO: 85 - protein, 34 aa, Artificial Sequence
  Synthetic Construct
  MISC_FEATURE (2)..(2): Xaa at position 2 is Aib
  MISC_FEATURE (6)..(6): Xaa at position 6 is alpha-methyl-Phe(2F)
  MISC_FEATURE (13)..(13): Xaa at position 13 is alpha-methyl-Leu
  MOD_RES (17)..(17): Lys at position 17 is chemically modified by conjugation of the epsilon-amino group of the Lys side chain with (2-[2-(2-amino-ethoxy)-ethoxy]-acetyl)2-(gamma-Glu)-CO-(CH2)18-CO 2H
  MISC_FEATURE (20)..(20): Xaa at position 20 is Aib
  MISC_FEATURE (24)..(24): Xaa at position 24 is D-Glu
  MOD_RES (34)..(34): Gly at position 34 is amidated
YXEGTXTSDHSIXLDEKAQXTFIXYLIEGGPSSG

SEQ ID NO: 86 - protein, 39 aa, Artificial Sequence
  Synthetic Construct
  MISC_FEATURE (2)..(2): Xaa at position 2 is Aib
  MISC_FEATURE (6)..(6): Xaa at position 6 is alpha-methyl-Phe(2F)
  MISC_FEATURE (13)..(13): Xaa at position 13 is alpha-methyl-Leu
  MOD_RES (17)..(17): Lys at position 17 is chemically modified by conjugation of the epsilon-amino group of the Lys side chain with (2-[2-(2-amino-ethoxy)-ethoxy]-acetyl)2-(gamma-Glu)-CO-(CH2)18-CO 2H
  MISC_FEATURE (20)..(20): Xaa at position 20 is Aib
  MISC_FEATURE (24)..(24): Xaa at position 24 is D-Glu
  MOD_RES (39)..(39): Ser at position 39 is amidated
YXEGTXTSDHSIXLDEKAQXTFIXYLIEGGPSSGAPPPS

SEQ ID NO: 87 - protein, 39 aa, Artificial Sequence; identical to SEQ ID NO: 86
  Synthetic Construct
  MISC_FEATURE (2)..(2): Xaa at position 2 is Aib
  MISC_FEATURE (6)..(6): Xaa at position 6 is alpha-methyl-Phe(2F)
  MISC_FEATURE (13)..(13): Xaa at position 13 is alpha-methyl-Leu
  MOD_RES (17)..(17): Lys at position 17 is chemically modified by conjugation of the epsilon-amino group of the Lys side chain with (2-[2-(2-amino-ethoxy)-ethoxy]-acetyl)2-(gamma-Glu)-CO-(CH2)16-CO 2H
  MISC_FEATURE (20)..(20): Xaa at position 20 is Aib
  MISC_FEATURE (24)..(24): Xaa at position 24 is D-Glu
  MOD_RES (39)..(39): Ser at position 39 is amidated

SEQ ID NO: 88 - protein, 39 aa, Artificial Sequence
  Synthetic Construct
  MISC_FEATURE (2)..(2): Xaa at position 2 is Aib
  MISC_FEATURE (6)..(6): Xaa at position 6 is alpha-methyl-Phe(2F)
  MISC_FEATURE (13)..(13): Xaa at position 13 is alpha-methyl-Leu
  MISC_FEATURE (16)..(16): Xaa at position 16 is Orn
  MOD_RES (17)..(17): Lys at position 17 is chemically modified by conjugation of the epsilon-amino group of the Lys side chain with (2-[2-(2-amino-ethoxy)-ethoxy]-acetyl)2-(gamma-Glu)-CO-(CH2)18-CO 2H
  MISC_FEATURE (20)..(20): Xaa at position 20 is Aib
  MISC_FEATURE (24)..(24): Xaa at position 24 is D-Glu
  MOD_RES (39)..(39): Ser at position 39 is amidated
YXEGTXTSDHSIXLDXKAQXTFIXYLIEGGPSSGAPPPS

SEQ ID NO: 89 - protein, 39 aa, Artificial Sequence; identical to SEQ ID NO: 88
  Synthetic Construct
  MISC_FEATURE (2)..(2): Xaa at position 2 is Aib
  MISC_FEATURE (6)..(6): Xaa at position 6 is alpha-methyl-Phe(2F)
  MISC_FEATURE (13)..(13): Xaa at position 13 is alpha-methyl-Leu
  MISC_FEATURE (16)..(16): Xaa at position 16 is Dab
  MOD_RES (17)..(17): Lys at position 17 is chemically modified by conjugation of the epsilon-amino group of the Lys side chain with (2-[2-(2-amino-ethoxy)-ethoxy]-acetyl)2-(gamma-Glu)-CO-(CH2)18-CO 2H
  MISC_FEATURE (20)..(20): Xaa at position 20 is a Aib
  MISC_FEATURE (24)..(24): Xaa at position 24 is D-Glu
  MOD_RES (39)..(39): Ser at position 39 is amidated

SEQ ID NO: 90 - protein, 39 aa, Artificial Sequence; identical to SEQ ID NO: 88
  Synthetic Construct
  MISC_FEATURE (2)..(2): Xaa at position 2 is Aib
  MISC_FEATURE (6)..(6): Xaa at position 6 is alpha-methyl-Phe(2F)
  MISC_FEATURE (13)..(13): Xaa at position 13 is alpha-methyl-Leu
  MISC_FEATURE (16)..(16): Xaa at position 16 is Dap
  MOD_RES (17)..(17): Lys at position 17 is chemically modified by conjugation of the epsilon-amino group of the Lys side chain with (2-[2-(2-amino-ethoxy)-ethoxy]-acetyl)2-(gamma-Glu)-CO-(CH2)18-CO 2H
  MISC_FEATURE (20)..(20): Xaa at position 20 is Aib
  MISC_FEATURE (24)..(24): Xaa at position 24 is D-Glu
  MOD_RES (39)..(39): Ser at position 39 is amidated

SEQ ID NO: 91 - protein, 39 aa, Artificial Sequence; identical to SEQ ID NO: 86
  Synthetic Construct
  MISC_FEATURE (2)..(2): Xaa at position 2 is Aib
  MISC_FEATURE (6)..(6): Xaa at position 6 is alpha-methyl-Phe(2F)
  MISC_FEATURE (13)..(13): Xaa at position 13 is alpha-methyl-Leu
  MOD_RES (17)..(17): Lys at position 17 is chemically modified by conjugation of the epsilon-amino group of the Lys side chain with (2-[2-(2-amino-ethoxy)-ethoxy]-acetyl)2-CO-(CH2)18-CO2H
  MISC_FEATURE (20)..(20): Xaa at position 20 is Aib
  MISC_FEATURE (24)..(24): Xaa at position 24 is D-Glu
  MOD_RES (39)..(39): Ser at position 39 is amidated

SEQ ID NO: 92 - protein, 39 aa, Artificial Sequence; identical to SEQ ID NO: 86
  Synthetic Construct
  MISC_FEATURE (2)..(2): Xaa at position 2 is Aib
  MISC_FEATURE (6)..(6): Xaa at position 6 is alpha-methyl-Phe(2F)
  MISC_FEATURE (13)..(13): Xaa at position 13 is alpha-methyl-Leu
  MOD_RES (17)..(17): Lys at position 17 is chemically modified by conjugation of the epsilon-amino group of the Lys side chain with (2-[2-(2-amino-ethoxy)-ethoxy]-acetyl)2-(epsilon-Lys)-CO-(CH2)16- CO2H
  MISC_FEATURE (20)..(20): Xaa at position 20 is Aib
  MISC_FEATURE (24)..(24): Xaa at position 24 is D-Glu
  MOD_RES (39)..(39): Ser at position 39 is amidated

SEQ ID NO: 93 - protein, 39 aa, Artificial Sequence
  Synthetic Construct
  MISC_FEATURE (2)..(2): Xaa at position 2 is Aib
  MISC_FEATURE (6)..(6): Xaa at position 6 is alpha-methyl-Phe(2F)
  MISC_FEATURE (13)..(13): Xaa at position 13 is alpha-methyl-Leu
  MOD_RES (17)..(17): Lys at position 17 is chemically modified by conjugation of the epsilon-amino group of the Lys side chain with (2-[2-(2-amino-ethoxy)-ethoxy]-acetyl)2-(gamma-Glu)-CO-(CH2)14-CO 2H
  MISC_FEATURE (20)..(20): Xaa at position 20 is Aib
  MISC_FEATURE (24)..(24): Xaa at position 24 is D-Glu
  MOD_RES (39)..(39): Ser at position 39 is amidated
YXEGTXTSDHSIXLDEKAQXHFIXYLIEGGPSSGAPPPS

SEQ ID NO: 94 - protein, 34 aa, Artificial Sequence
  Synthetic Construct
  MISC_FEATURE (2)..(2): Xaa at position 2 is Aib
  MISC_FEATURE (6)..(6): Xaa at position 6 is alpha-methyl-Phe(2F)
  MISC_FEATURE (13)..(13): Xaa at position 13 is alpha-methyl-Leu
  MOD_RES (17)..(17): Lys at position 17 is chemically modified by conjugation of the epsilon-amino group of the Lys side chain with (2-[2-(2-amino-ethoxy)-ethoxy]-acetyl)2-(gamma-Glu)-CO-(CH2)16-CO 2H
  MISC_FEATURE (20)..(20): Xaa at position 20 is Aib
  MISC_FEATURE (24)..(24): Xaa at position 24 is D-Glu
  MOD_RES (34)..(34): Gly at position 34 is amidated
YXEGTXTSDHSIXLDEKAQXHFIXYLIEGGPSSG

SEQ ID NO: 95 - protein, 30 aa, Artificial Sequence
  Synthetic Construct
  MISC_FEATURE (2)..(2): Xaa at position 2 is Aib
  MISC_FEATURE (6)..(6): Xaa at position 6 is alpha-methyl-Phe(2F)
  MISC_FEATURE (13)..(13): Xaa at position 13 is alpha-methyl-Leu
  MOD_RES (17)..(17): Lys at position 17 is chemically modified by conjugation of the epsilon-amino group of the Lys side chain with (2-[2-(2-amino-ethoxy)-ethoxy]-acetyl)2-(gamma-Glu)-CO-(CH2)16-CO 2H
  MISC_FEATURE (20)..(20): Xaa at position 20 is Aib
  MISC_FEATURE (24)..(24): Xaa at position 24 is D-Glu
  MOD_RES (30)..(30): Gly at position 30 is amidated
YXEGTXTSDHSIXLDEKAQXHFIXYLIEGG

SEQ ID NO: 96 - protein, 39 aa, Artificial Sequence
  Synthetic Construct
  MISC_FEATURE (2)..(2): Xaa at position 2 is Aib
  MISC_FEATURE (6)..(6): Xaa at position 6 is alpha-methyl-Phe(2F)
  MISC_FEATURE (10)..(10): Xaa at position 10 is 3Pal
  MISC_FEATURE (13)..(13): Xaa at position 13 is alpha-methyl-Leu
  MOD_RES (17)..(17): Lys at position 17 is chemically modified by conjugation of the epsilon-amino group of the Lys side chain with (2-[2-(2-amino-ethoxy)-ethoxy]-acetyl)2-(gamma-Glu)-CO-(CH2)18-CO 2H
  MISC_FEATURE (20)..(20): Xaa at position 20 is Aib
  MISC_FEATURE (24)..(24): Xaa at position 24 is D-Glu
  MOD_RES (39)..(39): Ser at position 39 is amidated
YXEGTXTSDXSIXLDEKAQXEFIXYLIEGGPSSGAPPPS

SEQ ID NO: 97 - protein, 39 aa, Artificial Sequence; identical to SEQ ID NO: 96
  Synthetic Construct
  MISC_FEATURE (2)..(2): Xaa at position 2 is Aib
  MISC_FEATURE (6)..(6): Xaa at position 6 is alpha-methyl-Phe(2F)
  MISC_FEATURE (10)..(10): Xaa at position 10 is 4Pal
  MISC_FEATURE (13)..(13): Xaa at position 13 is alpha-methyl-Leu
  MOD_RES (17)..(17): Lys at position 17 is chemically modified by conjugation of the epsilon-amino group of the Lys side chain with (2-[2-(2-amino-ethoxy)-ethoxy]-acetyl)2-(gamma-Glu)-CO-(CH2)18-CO 2H
  MISC_FEATURE (20)..(20): Xaa at position 20 is Aib
  MISC_FEATURE (24)..(24): Xaa at position 24 is D-Glu
  MOD_RES (39)..(39): Ser at position 39 is amidated

SEQ ID NO: 98 - protein, 39 aa, Artificial Sequence
  Synthetic Construct
  MISC_FEATURE (2)..(2): Xaa at position 2 is Aib
  MISC_FEATURE (6)..(6): Xaa at position 6 is alpha-methyl-Phe(2F)
  MISC_FEATURE (13)..(13): Xaa at position 13 is alpha-methyl-Leu
  MOD_RES (17)..(17): Lys at position 17 is chemically modified by conjugation of the epsilon-amino group of the Lys side chain with (2-[2-(2-amino-ethoxy)-ethoxy]-acetyl)2-(gamma-Glu)-CO-(CH2)18-CO 2H
  MISC_FEATURE (20)..(20): Xaa at position 20 is Aib
  MISC_FEATURE (24)..(24): Xaa at position 24 is D-Glu
  MOD_RES (39)..(39): Ser at position 39 is amidated
YXEGTXTSDLSIXLDEKAQXEFIXYLIEGGPSSGAPPPS

SEQ ID NO: 99 - protein, 39 aa, Artificial Sequence
  Synthetic Construct
  MISC_FEATURE (2)..(2): Xaa at position 2 is Aib
  MISC_FEATURE (6)..(6): Xaa at position 6 is alpha-methyl-Phe(2F)
  MISC_FEATURE (13)..(13): Xaa at position 13 is alpha-methyl-Leu
  MOD_RES (17)..(17): Lys at position 17 is chemically modified by conjugation of the epsilon-amino group of the Lys side chain with (2-[2-(2-amino-ethoxy)-ethoxy]-acetyl)2-(gamma-Glu)-CO-(CH2)18-CO 2H
  MISC_FEATURE (20)..(20): Xaa at position 20 is Aib
  MISC_FEATURE (24)..(24): Xaa at position 24 is D-Glu
  MOD_RES (39)..(39): Ser at position 39 is amidated
YXEGTXTSDQSIXLDEKAQXEFIXYLIEGGPSSGAPPPS

SEQ ID NO: 100 - protein, 39 aa, Artificial Sequence; identical to SEQ ID NO: 96
  Synthetic Construct
  MISC_FEATURE (2)..(2): Xaa at position 2 is Aib
  MISC_FEATURE (6)..(6): Xaa at position 6 is alpha-methyl-Phe(2F)
  MISC_FEATURE (10)..(10): Xaa at position 10 is 4Pal
  MISC_FEATURE (13)..(13): Xaa at position 13 is alpha-methyl-Leu
  MOD_RES (17)..(17): Lys at position 17 is chemically modified by conjugation of the epsilon-amino group of the Lys side chain with (2-[2-(2-amino-ethoxy)-ethoxy]-acetyl)2-(gamma-Glu)-CO-(CH2)18-CO 2H
  MISC_FEATURE (20)..(20): Xaa at position 20 is Aib
  MISC_FEATURE (24)..(24): Xaa at position 24 is Aib
  MOD_RES (39)..(39): Ser at position 39 is amidated

SEQ ID NO: 101 - protein, 34 aa, Artificial Sequence
  Synthetic Construct
  MISC_FEATURE (2)..(2): Xaa at position 2 is alpha-methyl-Pro
  MOD_RES (17)..(17): Lys at position 17 is chemically modified by conjugation of the epsilon-amino group of the Lys side chain with (2-[2-(2-amino-ethoxy)-ethoxy]-acetyl)2-(gamma-Glu)-CO-(CH2)16-CO 2H
  MOD_RES (34)..(34): Gly at position 34 is amidated
YXEGTFTSDYSILLDEKAQQAFIEYLIEGGPSSG

SEQ ID NO: 102 - protein, 39 aa, Artificial Sequence
  Synthetic Construct
  MISC_FEATURE (2)..(2): Xaa at position 2 is Aib
  MISC_FEATURE (6)..(6): Xaa at position 6 is alpha-methyl-Phe(2F)
  MISC_FEATURE (10)..(10): Xaa at position 10 is 4Pal
  MISC_FEATURE (13)..(13): Xaa at position 13 is alpha-methyl-Leu
  MOD_RES (17)..(17): Lys at position 17 is chemically modified by conjugation of the epsilon-amino group of the Lys side chain with (2-[2-(2-Amino-ethoxy)-ethoxy]-acetyl)-(gamma-Glu)-(2-[2-(2-Amino -ethoxy)-ethoxy]-acetyl)-CO-(CH2)18-CO2H
  MISC_FEATURE (20)..(20): Xaa at position 20 is Aib
  MISC_FEATURE (24)..(24): Xaa at position 24 is D-Glu
  MOD_RES (39)..(39): Ser at position 39 is amidated
YXEGTXTSDXSIXLDKKAQXEFIXYLIEGGPSSGAPPPS

SEQ ID NO: 103 - protein, 39 aa, Artificial Sequence; identical to SEQ ID NO: 102
  Synthetic Construct
  MISC_FEATURE (2)..(2): Xaa at position 2 is Aib
  MISC_FEATURE (6)..(6): Xaa at position 6 is alpha-methyl-Phe(2F)
  MISC_FEATURE (10)..(10): Xaa at position 10 is 4Pal
  MISC_FEATURE (13)..(13): Xaa at position 13 is alpha-methyl-Leu
  MOD_RES (17)..(17): Lys at position 17 is chemically modified by conjugation of the epsilon-amino group of the Lys side chain with (2-[2-(2-amino-ethoxy)-ethoxy]-acetyl)2-(gamma-Glu)-CO-(CH2)18-CO 2H
  MISC_FEATURE (20)..(20): Xaa at position 20 is Aib
  MISC_FEATURE (24)..(24): Xaa at position 24 is D-Glu
  MOD_RES (39)..(39): Ser at position 39 is amidated

SEQ ID NO: 104 - protein, 39 aa, Artificial Sequence; identical to SEQ ID NO: 96
  Synthetic Construct
  MISC_FEATURE (2)..(2): Xaa at position 2 is Aib
  MISC_FEATURE (6)..(6): Xaa at position 6 is alpha-methyl-Phe(2F)
  MISC_FEATURE (10)..(10): Xaa at position 10 is 4Pal
  MISC_FEATURE (13)..(13): Xaa at position 13 is alpha-methyl-Leu
  MOD_RES (17)..(17): Lys at position 17 is chemically modified by conjugation of the epsilon-amino group of the Lys side chain with (2-[2-(2-amino-ethoxy)-ethoxy]-acetyl)2-(gamma-Glu)-CO-(CH2)16-CO 2H
  MISC_FEATURE (20)..(20): Xaa at position 20 is Aib
  MISC_FEATURE (24)..(24): Xaa at position 24 is D-Glu
  MOD_RES (39)..(39): Ser at position 39 is amidated

SEQ ID NO: 105 - protein, 39 aa, Artificial Sequence; identical to SEQ ID NO: 96
  Synthetic Construct
  MISC_FEATURE (2)..(2): Xaa at position 2 is Aib
  MISC_FEATURE (6)..(6): Xaa at position 6 is alpha-methyl-Phe(2F)
  MISC_FEATURE (10)..(10): Xaa at position 10 is 4Pal
  MISC_FEATURE (13)..(13): Xaa at position 13 is alpha-methyl-Leu
  MOD_RES (17)..(17): Lys at position 17 is chemically modified by conjugation of the epsilon-amino group of the Lys side chain with (2-[2-(2-amino-ethoxy)-ethoxy]-acetyl)2-CO-(CH2)16-CO2H
  MISC_FEATURE (20)..(20): Xaa at position 20 is Aib
  MISC_FEATURE (24)..(24): Xaa at position 24 is D-Glu
  MOD_RES (39)..(39): Ser at position 39 is amidated

SEQ ID NO: 106 - protein, 39 aa, Artificial Sequence; identical to SEQ ID NO: 96
  Synthetic Construct
  MISC_FEATURE (2)..(2): Xaa at position 2 is Aib
  MISC_FEATURE (6)..(6): Xaa at position 6 is alpha-methyl-Phe(2F)
  MISC_FEATURE (10)..(10): Xaa at position 10 is 4Pal
  MISC_FEATURE (13)..(13): Xaa at position 13 is alpha-methyl-Leu
  MOD_RES (17)..(17): Lys at position 17 is chemically modified by conjugation of the epsilon-amino group of the Lys side chain with (2-[2-(2-amino-ethoxy)-ethoxy]-acetyl)2-CO-(CH2)18-CO2H
  MISC_FEATURE (20)..(20): Xaa at position 20 is Aib
  MISC_FEATURE (24)..(24): Xaa at position 24 is D-Glu
  MOD_RES (39)..(39): Ser at position 39 is amidated

SEQ ID NO: 107 - protein, 39 aa, Artificial Sequence; identical to SEQ ID NO: 96
  Synthetic Construct
  MISC_FEATURE (2)..(2): Xaa at position 2 is Aib
  MISC_FEATURE (6)..(6): Xaa at position 6 is alpha-methyl-Phe(2F)
  MISC_FEATURE (10)..(10): Xaa at position 10 is 4Pal
  MISC_FEATURE (13)..(13): Xaa at position 13 is alpha-methyl-Leu
  MOD_RES (17)..(17): Lys at position 17 is chemically modified by conjugation of the epsilon-amino group of the Lys side chain with (2-[2-(2-Amino-ethoxy)-ethoxy]-acetyl)2-(epsilon-Lys)-CO-(CH2)18- CO2H
  MISC_FEATURE (20)..(20): Xaa at position 20 is Aib
  MISC_FEATURE (24)..(24): Xaa at position 24 is D-Glu
  MOD_RES (39)..(39): Ser at position 39 is amidated

SEQ ID NO: 108 - protein, 39 aa, Artificial Sequence; identical to SEQ ID NO: 10
  Synthetic Construct
  MISC_FEATURE (2)..(2): Xaa at position 2 is Aib
  MISC_FEATURE (6)..(6): Xaa at position 6 is alpha-methyl-Phe(2F)
  MISC_FEATURE (13)..(13): Xaa at position 13 is alpha-methyl-Leu
  MOD_RES (17)..(17): Lys at position 17 is chemically modified by conjugation of the epsilon-amino group of the Lys side chain with (2-[2-(2-amino-ethoxy)-ethoxy]-acetyl)2-(gamma-Glu)-CO-(CH2)14-CO 2H
  MISC_FEATURE (20)..(20): Xaa at position 20 is Aib
  MISC_FEATURE (24)..(24): Xaa at position 24 is D-Glu
  MOD_RES (39)..(39): Ser at position 39 is amidated

SEQ ID NO: 109 - protein, 39 aa, Artificial Sequence; identical to SEQ ID NO: 11
  Synthetic Construct
  MISC_FEATURE (2)..(2): Xaa at position 2 is Aib
  MISC_FEATURE (6)..(6): Xaa at position 6 is alpha-methyl-Phe(2F)
  MISC_FEATURE (13)..(13): Xaa at position 13 is alpha-methyl-Leu
  MISC_FEATURE (16)..(16): Xaa at position 16 is Dab
  MOD_RES (17)..(17): Lys at position 17 is chemically modified by conjugation of the epsilon-amino group of the Lys side chain with (2-[2-(2-amino-ethoxy)-ethoxy]-acetyl)2-(gamma-Glu)-CO-(CH2)16-CO 2H
  MISC_FEATURE (20)..(20): Xaa at position 20 is Aib
  MISC_FEATURE (24)..(24): Xaa at position 24 is D-Glu
  MOD_RES (39)..(39): Ser at position 39 is amidated

SEQ ID NO: 110 - protein, 39 aa, Artificial Sequence; identical to SEQ ID NO: 11
  Synthetic Construct
  MISC_FEATURE (2)..(2): Xaa at position 2 is Aib
  MISC_FEATURE (6)..(6): Xaa at position 6 is alpha-methyl-Phe(2F)
  MISC_FEATURE (13)..(13): Xaa at position 13 is alpha-methyl-Leu
  MISC_FEATURE (16)..(16): Xaa at position 16 is Dap
  MOD_RES (17)..(17): Lys at position 17 is chemically modified by conjugation of the epsilon-amino group of the Lys side chain with (2-[2-(2-amino-ethoxy)-ethoxy]-acetyl)2-(gamma-Glu)-CO-(CH2)16-CO 2H
  MISC_FEATURE (20)..(20): Xaa at position 20 is Aib
  MISC_FEATURE (24)..(24): Xaa at position 24 is D-Glu
  MOD_RES (39)..(39): Ser at position 39 is amidated

SEQ ID NO: 111 - protein, 39 aa, Artificial Sequence
  Synthetic Construct
  MISC_FEATURE (2)..(2): Xaa at position 2 is Aib
  MISC_FEATURE (6)..(6): Xaa at position 6 is alpha-methyl-Phe(2F)
  MISC_FEATURE (13)..(13): Xaa at position 13 is alpha-methyl-Leu
  MOD_RES (17)..(17): Lys at position 17 is chemically modified by conjugation of the epsilon-amino group of the Lys side chain with (2-[2-(2-Amino-ethoxy)-ethoxy]-acetyl)-(gamma-Glu)-(2-[2-(2-Amino -ethoxy)-ethoxy]-acetyl)-CO-(CH2)18-CO2H
  MISC_FEATURE (20)..(20): Xaa at position 20 is Aib
  MISC_FEATURE (24)..(24): Xaa at position 24 is D-Glu
  MOD_RES (39)..(39): Ser at position 39 is amidated
YXEGTXTSDYSIXLDKKAQXEFIXYLIEGGPSSGAPPPS

SEQ ID NO: 112 - protein, 39 aa, Artificial Sequence; identical to SEQ ID NO: 111
  Synthetic Construct
  MISC_FEATURE (2)..(2): Xaa at position 2 is Aib
  MISC_FEATURE (6)..(6): Xaa at position 6 is alpha-methyl-Phe(2F)
  MISC_FEATURE (13)..(13): Xaa at position 13 is alpha-methyl-Leu
  MOD_RES (17)..(17): Lys at position 17 is chemically modified by conjugation of the epsilon-amino group of the Lys side chain with (2-[2-(2-amino-ethoxy)-ethoxy]-acetyl)2-(gamma-Glu)-CO-(CH2)18-CO 2H
  MISC_FEATURE (20)..(20): Xaa at position 20 is Aib
  MISC_FEATURE (24)..(24): Xaa at position 24 is D-Glu
  MOD_RES (39)..(39): Ser at position 39 is amidated

SEQ ID NO: 113 - protein, 39 aa, Artificial Sequence; identical to SEQ ID NO: 10
  Synthetic Construct
  MISC_FEATURE (2)..(2): Xaa at position 2 is Aib
  MISC_FEATURE (6)..(6): Xaa at position 6 is alpha-methyl-Phe
  MISC_FEATURE (13)..(13): Xaa at position 13 is alpha-methyl-Leu
  MOD_RES (17)..(17): Lys at position 17 is chemically modified by conjugation of the epsilon-amino group of the Lys side chain with (2-[2-(2-amino-ethoxy)-ethoxy]-acetyl)2-(gamma-Glu)-CO-(CH2)16-CO 2H
  MISC_FEATURE (20)..(20): Xaa at position 20 is Aib
  MISC_FEATURE (24)..(24): Xaa at position 24 is D-Glu
  MOD_RES (39)..(39): Ser at position 39 is amidated

SEQ ID NO: 114 - protein, 39 aa, Artificial Sequence; identical to SEQ ID NO: 10
  Synthetic Construct
  MISC_FEATURE (2)..(2): Xaa at position 2 is Aib
  MISC_FEATURE (6)..(6): Xaa at position 6 is alpha-methyl-Phe(2F)
  MISC_FEATURE (13)..(13): Xaa at position 13 is alpha-methyl-Leu
  MOD_RES (17)..(17): Lys at position 17 is chemically modified by conjugation of the epsilon-amino group of the Lys side chain with (2-[2-(2-amino-ethoxy)-ethoxy]-acetyl)2-CO-(CH2)16-CO2H
  MISC_FEATURE (20)..(20): Xaa at position 20 is Aib
  MISC_FEATURE (24)..(24): Xaa at position 24 is D-Glu
  MOD_RES (39)..(39): Ser at position 39 is amidated

SEQ ID NO: 115 - protein, 39 aa, Artificial Sequence; identical to SEQ ID NO: 10
  Synthetic Construct
  MISC_FEATURE (2)..(2): Xaa at position 2 is Aib
  MISC_FEATURE (6)..(6): Xaa at position 6 is alpha-methyl-Phe(2F)
  MISC_FEATURE (13)..(13): Xaa at position 13 is alpha-methyl-Leu
  MOD_RES (17)..(17): Lys at position 17 is chemically modified by conjugation of the epsilon-amino group of the Lys side chain with (2-[2-(2-amino-ethoxy)-ethoxy]-acetyl)2-CO-(CH2)18-CO2H
  MISC_FEATURE (20)..(20): Xaa at position 20 is Aib
  MISC_FEATURE (24)..(24): Xaa at position 24 is D-Glu
  MOD_RES (39)..(39): Ser at position 39 is amidated

SEQ ID NO: 116 - protein, 39 aa, Artificial Sequence; identical to SEQ ID NO: 10
  Synthetic Construct
  MISC_FEATURE (2)..(2): Xaa at position 2 is Aib
  MISC_FEATURE (6)..(6): Xaa at position 6 is alpha-methyl-Phe(2F)
  MISC_FEATURE (13)..(13): Xaa at position 13 is alpha-methyl-Leu
  MOD_RES (17)..(17): Lys at position 17 is chemically modified by conjugation of the epsilon-amino group of the Lys side chain with (2-[2-(2-amino-ethoxy)-ethoxy]-acetyl)2-(epsilon-Lys)-CO-(CH2)18- CO2H
  MISC_FEATURE (20)..(20): Xaa at position 20 is Aib
  MISC_FEATURE (24)..(24): Xaa at position 24 is D-Glu
  MOD_RES (39)..(39): Ser at position 39 is amidated

SEQ ID NO: 117 - protein, 39 aa, Artificial Sequence; identical to SEQ ID NO: 11
  Synthetic Construct
  MISC_FEATURE (2)..(2): Xaa at position 2 is Aib
  MISC_FEATURE (6)..(6): Xaa at position 6 is alpha-methyl-Phe(2F)
  MISC_FEATURE (13)..(13): Xaa at position 13 is alpha-methyl-Leu
  MISC_FEATURE (16)..(16): Xaa at position 16 is Dab
  MOD_RES (17)..(17): Lys at position 17 is chemically modified by conjugation of the epsilon-amino group of the Lys side chain with (2-[2-(2-amino-ethoxy)-ethoxy]-acetyl)2-(gamma-Glu)-CO-(CH2)18-CO 2H
  MISC_FEATURE (20)..(20): Xaa at position 20 is Aib
  MISC_FEATURE (24)..(24): Xaa at position 24 is D-Glu
  MOD_RES (39)..(39): Ser at position 39 is amidated

SEQ ID NO: 118 - protein, 39 aa, Artificial Sequence; identical to SEQ ID NO: 11
  Synthetic Construct
  MISC_FEATURE (2)..(2): Xaa at position 2 is Aib
  MISC_FEATURE (6)..(6): Xaa at position 6 is alpha-methyl-Phe(2F)
  MISC_FEATURE (13)..(13): Xaa at position 13 is alpha-methyl-Leu
  MISC_FEATURE (16)..(16): Xaa at position 16 is Dap
  MOD_RES (17)..(17): Lys at position 17 is chemically modified by conjugation of the epsilon-amino group of the Lys side chain with (2-[2-(2-amino-ethoxy)-ethoxy]-acetyl)2-(gamma-Glu)-CO-(CH2)18-CO 2H
  MISC_FEATURE (20)..(20): Xaa at position 20 is Aib
  MISC_FEATURE (24)..(24): Xaa at position 24 is D-Glu
  MOD_RES (39)..(39): Ser at position 39 is amidated

SEQ ID NO: 119 - protein, 34 aa, Artificial Sequence
  Synthetic Construct
  MISC_FEATURE (2)..(2): Xaa at position 2 is Aib
  MISC_FEATURE (6)..(6): Xaa at position 6 is alpha-methyl-Phe(2F)
  MISC_FEATURE (13)..(13): Xaa at position 13 is alpha-methyl-Leu
  MOD_RES (17)..(17): Lys at position 17 is chemically modified by conjugation of the epsilon-amino group of the Lys side chain with (2-[2-(2-amino-ethoxy)-ethoxy]-acetyl)2-(gamma-Glu)-CO-(CH2)16-CO 2H
  MISC_FEATURE (20)..(20): Xaa at position 20 is Aib
  MISC_FEATURE (24)..(24): Xaa at position 24 is D-Glu
  MOD_RES (34)..(34): Gly at position 34 is amidated
YXEGTXTSDYSIXLDEKAQXEFIXYLIEGGPSSG

SEQ ID NO: 120 - protein, 30 aa, Artificial Sequence
  Synthetic Construct
  MISC_FEATURE (2)..(2): Xaa at position 2 is Aib
  MISC_FEATURE (6)..(6): Xaa at position 6 is alpha-methyl-Phe(2F)
  MISC_FEATURE (13)..(13): Xaa at position 13 is alpha-methyl-Leu
  MOD_RES (17)..(17): Lys at position 17 is chemically modified by conjugation of the epsilon-amino group of the Lys side chain with (2-[2-(2-amino-ethoxy)-ethoxy]-acetyl)2-(gamma-Glu)-CO-(CH2)16-CO 2H
  MISC_FEATURE (20)..(20): Xaa at position 20 is Aib
  MISC_FEATURE (24)..(24): Xaa at position 24 is D-Glu
  MOD_RES (30)..(30): Gly at position 30 is amidated
YXEGTXTSDYSIXLDEKAQXEFIXYLIEGG

SEQ ID NO: 121 - protein, 39 aa, Artificial Sequence; identical to SEQ ID NO: 10
  Synthetic Construct
  MISC_FEATURE (2)..(2): Xaa at position 2 is Aib
  MISC_FEATURE (6)..(6): Xaa at position 6 is alpha-methyl-Phe(2F)
  MISC_FEATURE (13)..(13): Xaa at position 13 is alpha-methyl-Leu
  MOD_RES (17)..(17): Lys at position 17 is chemically modified by conjugation of the epsilon-amino group of the Lys side chain with (2-[2-(2-amino-ethoxy)-ethoxy]-acetyl)2-(gamma-Glu)-CO-(CH2)16-CO 2H
  MISC_FEATURE (20)..(20): Xaa at position 20 is Aib
  MISC_FEATURE (24)..(24): Xaa at position 24 is D-Glu
  MOD_RES (39)..(39): Ser at position 39 is amidated

SEQ ID NO: 122 - protein, 39 aa, Artificial Sequence
  Synthetic Construct
  MISC_FEATURE (2)..(2): Xaa at position 2 is Aib
  MISC_FEATURE (6)..(6): Xaa at position 6 is alpha-methyl-Phe(2F)
  MISC_FEATURE (13)..(13): Xaa at position 13 is alpha-methyl-Leu
  MOD_RES (17)..(17): Lys at position 17 is chemically modified by conjugation of the epsilon-amino group of the Lys side chain with (2-[2-(2-amino-ethoxy)-ethoxy]-acetyl)2-(gamma-Glu)-CO-(CH2)18-CO 2H
  MISC_FEATURE (20)..(20): Xaa at position 20 is Aib
  MISC_FEATURE (24)..(24): Xaa at position 24 is D-Glu
  MISC_FEATURE (25)..(25): Xaa at position 25 alpha-methyl-Tyr
  MOD_RES (39)..(39): Ser at position 39 is amidated
YXEGTXTSDYSIXLDEKAQXEFIXXLIEGGPSSGAPPPS

SEQ ID NO: 123 - protein, 39 aa, Artificial Sequence
  Synthetic Construct
  MISC_FEATURE (2)..(2): Xaa at position 2 is Aib
  MISC_FEATURE (6)..(6): Xaa at position 6 is alpha-methyl-Phe(2F)
  MISC_FEATURE (13)..(13): Xaa at position 13 is alpha-methyl-Leu
  MOD_RES (17)..(17): Lys at position 17 is chemically modified by conjugation of the epsilon-amino group of the Lys side chain with (2-[2-(2-amino-ethoxy)-ethoxy]-acetyl)2-(gamma-Glu)-CO-(CH2)18-CO 2H
  MISC_FEATURE (20)..(20): Xaa at position 20 is Aib
  MISC_FEATURE (25)..(25): Xaa at position 25 is alpha-methyl-Tyr
  MOD_RES (39)..(39): Ser at position 39 is amidated
YXEGTXTSDYSIXLDEKAQXEFIEXLIEGGPSSGAPPPS

SEQ ID NO: 124 - protein, 39 aa, Artificial Sequence; identical to SEQ ID NO: 10
  Synthetic Construct
  MISC_FEATURE (2)..(2): Xaa at position 2 is Aib
  MISC_FEATURE (6)..(6): Xaa at position 6 is alpha-methyl-Phe(2F)
  MISC_FEATURE (13)..(13): Xaa at position 13 is Aib
  MOD_RES (17)..(17): Lys at position 17 is chemically modified by conjugation of the epsilon-amino group of the Lys side chain with (2-[2-(2-amino-ethoxy)-ethoxy]-acetyl)2-(gamma-Glu)-CO-(CH2)18-CO 2H
  MISC_FEATURE (20)..(20): Xaa at position 20 is Aib
  MISC_FEATURE (24)..(24): Xaa at position 24 is D-Glu
  MOD_RES (39)..(39): Ser at position 39 is amidated

SEQ ID NO: 125 - protein, 39 aa, Artificial Sequence; identical to SEQ ID NO: 10
  Synthetic Construct
  MISC_FEATURE (2)..(2): Xaa at position 2 is Aib
  MISC_FEATURE (6)..(6): Xaa at position 6 is alpha-methyl-Phe
  MISC_FEATURE (13)..(13): Xaa at position 13 is Aib
  MOD_RES (17)..(17): Lys at position 17 is chemically modified by conjugation of the epsilon-amino group of the Lys side chain with (2-[2-(2-amino-ethoxy)-ethoxy]-acetyl)2-(gamma-Glu)-CO-(CH2)18-CO 2H
  MISC_FEATURE (20)..(20): Xaa at position 20 is Aib
  MISC_FEATURE (24)..(24): Xaa at position 24 is D-Glu
  MOD_RES (39)..(39): Ser at position 39 is amidated

SEQ ID NO: 126 - protein, 39 aa, Artificial Sequence
  Synthetic Construct
  MISC_FEATURE (2)..(2): Xaa at position 2 is Aib
  MISC_FEATURE (6)..(6): Xaa at position 6 is alpha-methyl-Phe(2F)
  MOD_RES (17)..(17): Lys at position 17 is chemically modified by conjugation of the epsilon-amino group of the Lys side chain with (2-[2-(2-amino-ethoxy)-ethoxy]-acetyl)2-(gamma-Glu)-CO-(CH2)18-CO 2H
  MISC_FEATURE (20)..(20): Xaa at position 20 is Aib
  MISC_FEATURE (24)..(24): Xaa at position 24 is D-Glu
  MOD_RES (39)..(39): Ser at position 39 is amidated
YXEGTXTSDYSILLDEKAQXEFIXYLIEGGPSSGAPPPS

SEQ ID NO: 127 - protein, 39 aa, Artificial Sequence; identical to SEQ ID NO: 10
  Synthetic Construct
  MISC_FEATURE (2)..(2): Xaa at position 2 is Aib
  MISC_FEATURE (6)..(6): Xaa at position 6 is alpha-methyl-Phe
  MISC_FEATURE (13)..(13): Xaa at position 13 is alpha-methyl-Leu
  MOD_RES (17)..(17): Lys at position 17 is chemically modified by conjugation of the epsilon-amino group of the Lys side chain with (2-[2-(2-amino-ethoxy)-ethoxy]-acetyl)2-(gamma-Glu)-CO-(CH2)18-CO 2H
  MISC_FEATURE (20)..(20): Xaa at position 20 is Aib
  MISC_FEATURE (24)..(24): Xaa at position 24 is D-Glu
  MOD_RES (39)..(39): Ser at position 39 is amidated

SEQ ID NO: 128 - protein, 34 aa, Artificial Sequence
  Synthetic Construct
  MISC_FEATURE (2)..(2): Xaa at position 2 is Aib
  MISC_FEATURE (6)..(6): Xaa at position 6 is alpha-methyl-Phe
  MISC_FEATURE (13)..(13): Xaa at position 13 is alpha-methyl-Leu
  MOD_RES (17)..(17): Lys at position 17 is chemically modified by conjugation of the epsilon-amino group of the Lys side chain with (2-[2-(2-amino-ethoxy)-ethoxy]-acetyl)2-(gamma-Glu)-CO-(CH2)18-CO 2H
  MISC_FEATURE (20)..(20): Xaa at position 20 is Aib
  MISC_FEATURE (24)..(24): Xaa at position 24 is D-Glu
  MOD_RES (34)..(34): Gly at position 34 is amidated
YXEGTXTSDYSIXLDKKAQXEFIXYLIEGGPSSG

SEQ ID NO: 129 - protein, 39 aa, Artificial Sequence
  Synthetic Construct
  MISC_FEATURE (2)..(2): Xaa at position 2 is Aib
  MISC_FEATURE (6)..(6): Xaa at position 6 is alpha-methyl-Phe(2F)
  MISC_FEATURE (13)..(13): Xaa at position 13 is alpha-methyl-Leu
  MOD_RES (17)..(17): Lys at position 17 is chemically modified by conjugation of the epsilon-amino group of the Lys side chain with (2-[2-(2-amino-ethoxy)-ethoxy]-acetyl)2-(gamma-Glu)-CO-(CH2)18-CO 2H
  MISC_FEATURE (20)..(20): Xaa at position 20 is Aib
  MISC_FEATURE (24)..(24): Xaa at position 24 is D-Glu
  MOD_RES (39)..(39): Ser at position 39 is amidated
YXEGTXTSDYSIXLDHKAQXEFIXYLIEGGPSSGAPPPS

SEQ ID NO: 130 - protein, 39 aa, Artificial Sequence
  Synthetic Construct
  MISC_FEATURE (2)..(2): Xaa at position 2 is Aib
  MISC_FEATURE (6)..(6): Xaa at position 6 is alpha-methyl-Phe(2F)
  MISC_FEATURE (10)..(10): Xaa at position 10 is 4Pal
  MISC_FEATURE (13)..(13): Xaa at position 13 is alpha-methyl-Leu
  MISC_FEATURE (16)..(16): Xaa at position 16 is Dab
  MOD_RES (17)..(17): Lys at position 17 is chemically modified by conjugation of the epsilon-amino group of the Lys side chain with (2-[2-(2-amino-ethoxy)-ethoxy]-acetyl)2-(gamma-Glu)-CO-(CH2)16-CO 2H
  MISC_FEATURE (20)..(20): Xaa at position 20 is Aib
  MISC_FEATURE (24)..(24): Xaa at position 24 is D-Glu
  MOD_RES (39)..(39): Ser at position 39 is amidated
YXEGTXTSDXSIXLDXKAQXEFIXYLIEGGPSSGAPPPS

SEQ ID NO: 131 - protein, 39 aa, Artificial Sequence
  Synthetic Construct
  MISC_FEATURE (2)..(2): Xaa at position 2 is Aib
  MISC_FEATURE (6)..(6): Xaa at position 6 is alpha-methyl-Phe(2F)
  MISC_FEATURE (13)..(13): Xaa at position 13 is alpha-methyl-Leu
  MISC_FEATURE (16)..(16): Xaa at position 16 is Orn
  MOD_RES (17)..(17): Lys at position 17 is chemically modified by conjugation of the epsilon-amino group of the Lys side chain with (2-[2-(2-amino-ethoxy)-ethoxy]-acetyl)2-(gamma-Glu)-CO-(CH2)16-CO 2H
  MISC_FEATURE (20)..(20): Xaa at position 20 is Aib
  MISC_FEATURE (24)..(24): Xaa at position 24 is D-Glu
  MISC_FEATURE (25)..(25): Xaa at position 25 is alpha-methyl-Tyr
  MOD_RES (39)..(39): Ser at position 39 is amidated
YXEGTXTSDYSIXLDXKAQXEFIXXLIEGGPSSGAPPPS

SEQ ID NO: 132 - protein, 39 aa, Artificial Sequence
  Synthetic Construct
  MISC_FEATURE (2)..(2): Xaa at position 2 is Aib
  MISC_FEATURE (6)..(6): Xaa at position 6 is alpha-methyl-Phe(2F)
  MISC_FEATURE (13)..(13): Xaa at position 13 is alpha-methyl-Leu
  MISC_FEATURE (16)..(16): Xaa at position 16 is Orn
  MOD_RES (17)..(17): Lys at position 17 is chemically modified by conjugation of the epsilon-amino group of the Lys side chain with (2-[2-(2-amino-ethoxy)-ethoxy]-acetyl)2-(gamma-Glu)-CO-(CH2)16-CO 2H
  MISC_FEATURE (20)..(20): Xaa at position 20 is Aib
  MISC_FEATURE (24)..(24): Xaa at position 24 is D-Glu
  MISC_FEATURE (25)..(25): Xaa at position 25 is alpha-methyl-Tyr
  MOD_RES (39)..(39): Ser at position 39 is amidated
YXEGTXTSDLSIXLDXKAQXEFIXXLIEGGPSSGAPPPS

SEQ ID NO: 133 - protein, 39 aa, Artificial Sequence
  Synthetic Construct
  MISC_FEATURE (2)..(2): Xaa at position 2 is Aib
  MISC_FEATURE (6)..(6): Xaa at position 6 is alpha-methyl-Phe(2F)
  MISC_FEATURE (10)..(10): Xaa at position 10 is 4Pal
  MISC_FEATURE (13)..(13): Xaa at position 13 is alpha-methyl-Leu
  MISC_FEATURE (16)..(16): Xaa at position 16 is Orn
  MOD_RES (17)..(17): Lys at position 17 is chemically modified by conjugation of the epsilon-amino group of the Lys side chain with (2-[2-(2-amino-ethoxy)-ethoxy]-acetyl)2-(gamma-Glu)-CO-(CH2)16-CO 2H
  MISC_FEATURE (20)..(20): Xaa at position 20 is Aib
  MISC_FEATURE (24)..(24): Xaa at position 24 is D-Glu
  MISC_FEATURE (25)..(25): Xaa at position 25 is alpha-methyl-Tyr
  MOD_RES (39)..(39): Ser at position 39 is amidated
YXEGTXTSDXSIXLDXKAQXTFIXXLIEGGPSSGAPPPS

SEQ ID NO: 134 - protein, 39 aa, Artificial Sequence
  Synthetic Construct
  MISC_FEATURE (2)..(2): Xaa at position 2 is Aib
  MISC_FEATURE (6)..(6): Xaa at position 6 is alpha-methyl-Phe(2F)
  MISC_FEATURE (13)..(13): Xaa at position 13 is alpha-methyl-Leu
  MISC_FEATURE (16)..(16): Xaa at position 16 is Orn
  MOD_RES (17)..(17): Lys at position 17 is chemically modified by conjugation of the epsilon-amino group of the Lys side chain with (2-[2-(2-amino-ethoxy)-ethoxy]-acetyl)2-(gamma-Glu)-CO-(CH2)16-CO 2H
  MISC_FEATURE (20)..(20): Xaa at position 20 is Aib
  MISC_FEATURE (24)..(24): Xaa at position 24 is D-Glu
  MISC_FEATURE (25)..(25): Xaa at position 25 is alpha-methyl-Tyr
  MOD_RES (39)..(39): Ser at position 39 is amidated
YXEGTXTSDVSIXLDXKAQXTFIXXLIEGGPSSGAPPPS

SEQ ID NO: 135 - protein, 39 aa, Artificial Sequence
  Synthetic Construct
  MISC_FEATURE (2)..(2): Xaa at position 2 is Aib
  MISC_FEATURE (6)..(6): Xaa at position 6 is alpha-methyl-Phe(2F)
  MISC_FEATURE (13)..(13): Xaa at position 13 is alpha-methyl-Leu
  MISC_FEATURE (16)..(16): Xaa at position 16 is Orn
  MOD_RES (17)..(17): Lys at position 17 is chemically modified by conjugation of the epsilon-amino group of the Lys side chain with (2-[2-(2-amino-ethoxy)-ethoxy]-acetyl)2-(gamma-Glu)-CO-(CH2)16-CO 2H
  MISC_FEATURE (20)..(20): Xaa at position 20 is Aib
  MISC_FEATURE (24)..(24): Xaa at position 24 is D-Glu
  MISC_FEATURE (25)..(25): Xaa at position 25 is alpha-methyl-Tyr
  MOD_RES (39)..(39): Ser at position 39 is amidated
YXEGTXTSDVSIXLDXKAQXAFIXXLIEGGPSSGAPPPS

SEQ ID NO: 136 - protein, 39 aa, Artificial Sequence
  Synthetic Construct
  MISC_FEATURE (2)..(2): Xaa at position 2 is Aib
  MISC_FEATURE (6)..(6): Xaa at position 6 is alpha-methyl-Phe(2F)
  MISC_FEATURE (13)..(13): Xaa at position 13 is alpha-methyl-Leu
  MISC_FEATURE (16)..(16): Xaa at position 16 is Orn
  MOD_RES (17)..(17): Lys at position 17 is chemically modified by conjugation of the epsilon-amino group of the Lys side chain with (2-[2-(2-amino-ethoxy)-ethoxy]-acetyl)2-(gamma-Glu)-CO-(CH2)16-CO 2H
  MISC_FEATURE (20)..(20): Xaa at position 20 is Aib
  MISC_FEATURE (24)..(24): Xaa at position 24 is D-Glu
  MISC_FEATURE (25)..(25): Xaa at position 25 is alpha-methyl-Tyr
  MOD_RES (39)..(39): Ser at position 39 is amidated
YXEGTXTSDLSIXLDXKAQXTFIXXLIEGGPSSGAPPPS

SEQ ID NO: 137 - protein, 39 aa, Artificial Sequence
  Synthetic Construct
  MISC_FEATURE (2)..(2): Xaa at position 2 is Aib
  MISC_FEATURE (6)..(6): Xaa at position 6 is alpha-methyl-Phe(2F)
  MISC_FEATURE (13)..(13): Xaa at position 13 is alpha-methyl-Leu
  MISC_FEATURE (16)..(16): Xaa at position 16 is Orn
  MOD_RES (17)..(17): Lys at position 17 is chemically modified by conjugation of the epsilon-amino group of the Lys side chain with (2-[2-(2-amino-ethoxy)-ethoxy]-acetyl)2-(gamma-Glu)-CO-(CH2)16-CO 2H
  MISC_FEATURE (20)..(20): Xaa at position 20 is Aib
  MISC_FEATURE (24)..(24): Xaa at position 24 is D-Glu
  MISC_FEATURE (25)..(25): Xaa at position 25 is alpha-methyl-Tyr
  MOD_RES (39)..(39): Ser at position 39 is amidated
YXEGTXTSDLSIXLDXKAQXAFIXXLIEGGPSSGAPPPS

SEQ ID NO: 138 - protein, 39 aa, Artificial Sequence
  Synthetic Construct
  MISC_FEATURE (2)..(2): Xaa at position 2 is Aib
  MISC_FEATURE (6)..(6): Xaa at position 6 is alpha-methyl-Phe(2F)
  MISC_FEATURE (13)..(13): Xaa at position 13 is alpha-methyl-Leu
  MISC_FEATURE (16)..(16): Xaa at position 16 is Orn
  MOD_RES (17)..(17): Lys at position 17 is chemically modified by conjugation of the epsilon-amino group of the Lys side chain with (2-[2-(2-amino-ethoxy)-ethoxy]-acetyl)2-(gamma-Glu)-CO-(CH2)16-CO 2H
  MISC_FEATURE (20)..(20): Xaa at position 20 is Aib
  MISC_FEATURE (24)..(24): Xaa at position 24 is D-Glu
  MISC_FEATURE (25)..(25): Xaa at position 25 is alpha-methyl-Tyr
  MOD_RES (39)..(39): Ser at position 39 is amidated
YXEGTXTSDASIXLDXKAQXAFIXXLIEGGPSSGAPPPS

SEQ ID NO: 139 - protein, 39 aa, Artificial Sequence; identical to SEQ ID NO: 11
  Synthetic Construct
  MISC_FEATURE (2)..(2): Xaa at position 2 is Aib
  MISC_FEATURE (6)..(6): Xaa at position 6 is alpha-methyl-Phe(2F)
  MISC_FEATURE (13)..(13): Xaa at position 13 is Aib
  MISC_FEATURE (16)..(16): Xaa at position 16 is Orn
  MOD_RES (17)..(17): Lys at position 17 is chemically modified by conjugation of the epsilon-amino group of the Lys side chain with (2-[2-(2-amino-ethoxy)-ethoxy]-acetyl)2-(gamma-Glu)-CO-(CH2)16-CO 2H
  MISC_FEATURE (20)..(20): Xaa at position 20 is Aib
  MISC_FEATURE (24)..(24): Xaa at position 24 is D-Glu
  MOD_RES (39)..(39): Ser at position 39 is amidated

SEQ ID NO: 140 - protein, 39 aa, Artificial Sequence
  Synthetic Construct
  MISC_FEATURE (2)..(2): Xaa at position 2 is Aib
  MISC_FEATURE (6)..(6): Xaa at position 6 is alpha-methyl-Phe(2F)
  MISC_FEATURE (16)..(16): Xaa at position 16 is Orn
  MOD_RES (17)..(17): Lys at position 17 is chemically modified by conjugation of the epsilon-amino group of the Lys side chain with (2-[2-(2-amino-ethoxy)-ethoxy]-acetyl)2-(gamma-Glu)-CO-(CH2)16-CO 2H
  MISC_FEATURE (20)..(20): Xaa at position 20 is Aib
  MISC_FEATURE (24)..(24): Xaa at position 24 is D-Glu
  MOD_RES (39)..(39): Ser at position 39 is amidated
YXEGTXTSDYSILLDXKAQXEFIXYLIEGGPSSGAPPPS

SEQ ID NO: 141 - protein, 39 aa, Artificial Sequence; identical to SEQ ID NO: 11
  Synthetic Construct
  MISC_FEATURE (2)..(2): Xaa at position 2 is Aib
  MISC_FEATURE (6)..(6): Xaa at position 6 is alpha-methyl-Phe(2F)
  MISC_FEATURE (13)..(13): Xaa at position 13 is Nle
  MISC_FEATURE (16)..(16): Xaa at position 16 is Orn
  MOD_RES (17)..(17): Lys at position 17 is chemically modified by conjugation of the epsilon-amino group of the Lys side chain with (2-[2-(2-amino-ethoxy)-ethoxy]-acetyl)2-(gamma-Glu)-CO-(CH2)16-CO 2H
  MISC_FEATURE (20)..(20): Xaa at position 20 is Aib
  MISC_FEATURE (24)..(24): Xaa at position 24 is D-Glu
  MOD_RES (39)..(39): Ser at position 39 is amidated

SEQ ID NO: 142 - protein, 39 aa, Artificial Sequence; identical to SEQ ID NO: 11
  Synthetic Construct
  MISC_FEATURE (2)..(2): Xaa at position 2 is Aib
  MISC_FEATURE (6)..(6): Xaa at position 6 is alpha-methyl-Phe(2F)
  MISC_FEATURE (13)..(13): Xaa at position 13 is Aib
  MISC_FEATURE (16)..(16): Xaa at position 16 is Orn
  MOD_RES (17)..(17): Lys at position 17 is chemically modified by conjugation of the epsilon-amino group of the Lys side chain with (2-[2-(2-amino-ethoxy)-ethoxy]-acetyl)2-(gamma-Glu)-CO-(CH2)18-CO 2H
  MISC_FEATURE (20)..(20): Xaa at position 20 is Aib
  MISC_FEATURE (24)..(24): Xaa at position 24 is D-Glu
  MOD_RES (39)..(39): Ser at position 39 is amidated

SEQ ID NO: 143 - protein, 39 aa, Artificial Sequence
  Synthetic Construct
  MISC_FEATURE (2)..(2): Xaa at position 2 is Aib
  MISC_FEATURE (6)..(6): Xaa at position 6 is alpha-methyl-Phe(2F)
  MISC_FEATURE (10)..(10): Xaa at position 10 is 4Pal
  MISC_FEATURE (13)..(13): Xaa at position 13 is alpha-methyl-Leu
  MISC_FEATURE (16)..(16): Xaa at position 16 is Orn
  MOD_RES (17)..(17): Lys at position 17 is chemically modified by conjugation of the epsilon-amino group of the Lys side chain with (2-[2-(2-amino-ethoxy)-ethoxy]-acetyl)2-(epsilon-Lys)-CO-(CH2)18- CO2H
  MISC_FEATURE (20)..(20): Xaa at position 20 is Aib
  MISC_FEATURE (24)..(24): Xaa at position 24 is D-Glu
  MISC_FEATURE (25)..(25): Xaa at position 25 is alpha-methyl-Tyr
  MOD_RES (39)..(39): Ser at position 39 is amidated
YXEGTXTSDXSIXLDXKAQXAFIXXLIEGGPSSGAPPPS

SEQ ID NO: 144 - protein, 34 aa, Artificial Sequence
  Synthetic Construct
  MISC_FEATURE (2)..(2): Xaa at position 2 is Aib
  MISC_FEATURE (6)..(6): Xaa at position 6 is alpha-methyl-Phe(2F)
  MISC_FEATURE (10)..(10): Xaa at position 10 is 4Pal
  MISC_FEATURE (13)..(13): Xaa at position 13 is alpha-methyl-Leu
  MISC_FEATURE (16)..(16): Xaa at position 16 is Orn
  MOD_RES (17)..(17): Lys at position 17 is chemically modified by conjugation of the epsilon-amino group of the Lys side chain with (2-[2-(2-amino-ethoxy)-ethoxy]-acetyl)2-(gamma-Glu)-CO-(CH2)16-CO 2H
  MISC_FEATURE (20)..(20): Xaa at position 20 is Aib
  MISC_FEATURE (24)..(24): Xaa at position 24 is D-Glu
  MISC_FEATURE (25)..(25): Xaa at position 25 is alpha-methyl-Tyr
  MOD_RES (34)..(34): Gly at position 34 is amidated
YXEGTXTSDXSIXLDXKAQXEFIXXLIEGGPSSG

SEQ ID NO: 145 - protein, 30 aa, Artificial Sequence
  Synthetic Construct
  MISC_FEATURE (2)..(2): Xaa at position 2 is Aib
  MISC_FEATURE (6)..(6): Xaa at position 6 is alpha-methyl-Phe(2F)
  MISC_FEATURE (10)..(10): Xaa at position 10 is 4Pal
  MISC_FEATURE (13)..(13): Xaa at position 13 is alpha-methyl-Leu
  MISC_FEATURE (16)..(16): Xaa at position 13 is Orn
  MOD_RES (17)..(17): Lys at position 17 is chemically modified by conjugation of the epsilon-amino group of the Lys side chain with (2-[2-(2-amino-ethoxy)-ethoxy]-acetyl)2-(gamma-Glu)-CO-(CH2)16-CO 2H
  MISC_FEATURE (20)..(20): Xaa at position 20 is Aib
  MISC_FEATURE (24)..(24): Xaa at position 24 is D-Glu
  MISC_FEATURE (25)..(25): Xaa at position 25 is alpha-methyl-Tyr
  MOD_RES (30)..(30): Gly at position 30 is amidated
YXEGTXTSDXSIXLDXKAQXEFIXXLIEGG